European Patent Application EP 4 803 139 A2, published September 9, 2026. Title: METHODS OF TREATING OR PREVENTING CHOLESTEROL RELATED DISORDERS. Applicant: AMGEN, INC. The sequence listing filed with the application follows.

SEQUENCE LISTING (589 sequences)

SEQ ID NO: 1 - protein, 662 aa, Homo sapiens
QEDEDGDYEELVLALRSEEDGLAEAPEHGTTATFHRCAKDPWRLPGTYVVVLKEETHLSQSERTARRLQAQAARRGYLTKILHVFHGLLPGFLVKMSGDLLELALKLPHVDYIEEDSSVFAQSIPWNLERITPPRYRADEYQPPDGGSLVEVYLLDTSIQSDHREIEGRVMVTDFENVPEEDGTRFHRQASKCDSHGTHLAGVVSGRDAGVAKGASMRSLRVLNCQGKGTVSGTLIGLEFIRKSQLVQPVGPLVVLLPLAGGYSRVLNAACQRLARAGVVLVTAAGNFRDDACLYSPASAPEVITVGATNAQDQPVTLGTLGTNFGRCVDLFAPGEDIIGASSDCSTCFVSQSGTSQAAAHVAGIAAMMLSAEPELTLAELRQRLIHFSAKDVINEAWFPEDQRVLTPNLVAALPPSTHGAGWQLFCRTVWSAHSGPTRMATAIARCAPDEELLSCSSFSRSGKRRGERMEAQGGKLVCRAHNAFGGEGVYAIARCCLLPQANCSVHTAPPAEASMGTRVHCHQQGHVLTGCSSHWEVEDLGTHKPPVLRPRGQPNQCVGHREASIHASCCHAPGLECKVKEHGIPAPQGQVTVACEEGWTLTGCSALPGTSHVLGAYAVDNTCVVRSRDVSTTGSTSEEAVTAVAICCRSRHLAQASQELQ

SEQ ID NO: 2 - DNA, 2076 bp, Homo sapiens
  source 1..2076: mol_type = unassigned DNA
atgggcaccgtcagctccaggcggtcctggtggccgctgccactgctgctgctgctgctgctgctcctgggtcccgcgggcgcccgtgcgcaggaggacgaggacggcgactacgaggagctggtgctagccttgcgctccgaggaggacggcctggccgaagcacccgagcacggaaccacagccaccttccaccgctgcgccaaggatccgtggaggttgcctggcacctacgtggtggtgctgaaggaggagacccacctctcgcagtcagagcgcactgcccgccgcctgcaggcccaggctgcccgccggggatacctcaccaagatcctgcatgtcttccatggccttcttcctggcttcctggtgaagatgagtggcgacctgctggagctggccttgaagttgccccatgtcgactacatcgaggaggactcctctgtctttgcccagagcatcccgtggaacctggagcggattacccctccgcggtaccgggcggatgaataccagccccccgacggaggcagcctggtggaggtgtatctcctagacaccagcatacagagtgaccaccgggaaatcgagggcagggtcatggtcaccgacttcgagaatgtgcccgaggaggacgggacccgcttccacagacaggccagcaagtgtgacagtcatggcacccacctggcaggggtggtcagcggccgggatgccggcgtggccaagggtgccagcatgcgcagcctgcgcgtgctcaactgccaagggaagggcacggttagcggcaccctcataggcctggagtttattcggaaaagccagctggtccagcctgtggggccactggtggtgctgctgcccctggcgggtgggtacagccgcgtcctcaacgccgcctgccagcgcctggcgagggctggggtcgtgctggtcaccgctgccggcaacttccgggacgatgcctgcctctactccccagcctcagctcccgaggtcatcacagttggggccaccaatgcccaggaccagccggtgaccctggggactttggggaccaactttggccgctgtgtggacctctttgccccaggggaggacatcattggtgcctccagcgactgcagcacctgctttgtgtcacagagtgggacatcacaggctgctgcccacgtggctggcattgcagccatgatgctgtctgccgagccggagctcaccctggccgagttgaggcagagactgatccacttctctgccaaagatgtcatcaatgaggcctggttccctgaggaccagcgggtactgacccccaacctggtggccgccctgccccccagcacccatggggcaggttggcagctgttttgcaggactgtgtggtcagcacactcggggcctacacggatggccacagccatcgcccgctgcgccccagatgaggagctgctgagctgctccagtttctccaggagtgggaagcggcggggcgagcgcatggaggcccaagggggcaagctggtctgccgggcccacaacgcttttgggggtgagggtgtctacgccattgccaggtgctgcctgctaccccaggccaactgcagcgtccacacagctccaccagctgaggccagcatggggacccgtgtccactgccaccaacagggccacgtcctcacaggctgcagctcccactgggaggtggaggaccttggcacccacaagccgcctgtgctgaggccacgaggtcagcccaaccagtgcgtgggccacagggaggccagcatccacgcttcctgctgccatgccccaggtctggaatgcaaagtcaaggagcatggaatcccggcccctcaggggcaggtgaccgtggcctgcgaggagggctggaccctgactggctgcagcgccctccctgggacctcccacgtcctgggggcctacgccgtagacaacacgtgtgtagtcaggagccgggacgtcagcactacaggcagcaccagcgaagaggccgtgacagccgttgccatctgctgccggagccggcacctggcgcaggcctcccaggagctccag

SEQ ID NO: 3 - protein, 692 aa, Homo sapiens
MGTVSSRRSWWPLPLLLLLLLLLGPAGARAQEDEDGDYEELVLALRSEEDGLAEAPEHGTTATFHRCAKDPWRLPGTYVVVLKEETHLSQSERTARRLQAQAARRGYLTKILHVFHGLLPGFLVKMSGDLLELALKLPHVDYIEEDSSVFAQSIPWNLERITPPRYRADEYQPPDGGSLVEVYLLDTSIQSDHREIEGRVMVTDFENVPEEDGTRFHRQASKCDSHGTHLAGVVSGRDAGVAKGASMRSLRVLNCQGKGTVSGTLIGLEFIRKSQLVQPVGPLVVLLPLAGGYSRVLNAACQRLARAGVVLVTAAGNFRDDACLYSPASAPEVITVGATNAQDQPVTLGTLGTNFGRCVDLFAPGEDIIGASSDCSTCFVSQSGTSQAAAHVAGIAAMMLSAEPELTLAELRQRLIHFSAKDVINEAWFPEDQRVLTPNLVAALPPSTHGAGWQLFCRTVWSAHSGPTRMATAIARCAPDEELLSCSSFSRSGKRRGERMEAQGGKLVCRAHNAFGGEGVYAIARCCLLPQANCSVHTAPPAEASMGTRVHCHQQGHVLTGCSSHWEVEDLGTHKPPVLRPRGQPNQCVGHREASIHASCCHAPGLECKVKEHGIPAPQGQVTVACEEGWTLTGCSALPGTSHVLGAYAVDNTCVVRSRDVSTTGSTSEEAVTAVAICCRSRHLAQASQELQ

SEQ ID NO: 4 - protein, 112 aa, Homo sapiens
DIVMTQSPLSLPVTPGEPASISCRSSQSLLHSNGYNYLDWYLQKPGQSPQLLIYLGSNRASGVPDRFSGSGSGTDFTLKISRVEAEDVGVYYCMQALQTPFTFGPGTKVDIK

SEQ ID NO: 5 - protein, 112 aa, Homo sapiens
DIVMTQSPLSLSVTPGEPPSISCRSSQSLLHSNGYNFLNWYLQKPGQSPQLLIYLGSHRASGVPDRFSGSGSGTDFTLEISRVEAEDVGVYYCMQVLQTPFTFGPGTKVDIK

SEQ ID NO: 6 - protein, 107 aa, Homo sapiens [sequence omitted]

SEQ ID NO: 7 - protein, 107 aa, Homo sapiens
DIQMTQSPSSLSASVGDRVTITCRASQRISNYLSWYLQKPGIAPKLLIYAASSLQSGVPSRFSGSGSGTDFTLTISSLQSEDFATYYCQQSYSTPLIFGGGTKVEIK

SEQ ID NO: 8 - protein, 107 aa, Homo sapiens
DIQMTQSPSSLSASVGDRVTITCRASQSISSYLNWYQQKPGKAPKLLIYAASSLQSGVPSRFSGSGSGTDFTLTISSLQPEDFATYYCQQSYSTPITFGQGTRLEIK

SEQ ID NO: 9 - protein, 107 aa, Homo sapiens
DILMTQSPSSLSASVGDRVTITCRASQSISSYLNWYQQKPGKAPKVLIYAASSLQSGVPSRFSGSGSGTDFTLTINSLQPEDFATYYCQQSYSSPITFGQGTRLEIK

SEQ ID NO: 10 - protein, 107 aa, Homo sapiens
DIQMTQSPSSLSASVGDRVTITCRASQSISIYLNWYQQKPGKAPYLLIYAAASLQSGVPSRFSGSGSGTDFTLTISSLQPEDFATYYCQQSYSAPITFGQGTRLEIK

SEQ ID NO: 11 - protein, 111 aa, Homo sapiens
QSVLTQPPSVSGAPGQRVTISCTGSSSNIGAGYDVHWYQQLPGTAPKLLIYGNSNRPSGVPDRFSGSKSGTSASLAITGLQAEDEADYYCQSYDSSLSGSVFGGGTKLTVL

SEQ ID NO: 12 - protein, 111 aa, Homo sapiens
QSVLTQPPSVSGAPGQRVTISCTGSSSNIGAGYDVHWYQQLPGTAPKLLISGNSNRPSGVPDRFSGSKSGTSASLAITGLQAEDEADYYCQSYDSSLSGSVFGGGTKLTVL

SEQ ID NO: 13 - protein, 111 aa, Homo sapiens
QSVLTQPPSVSGAPGQRVTISCTGSSSNIGAHYDVHWYQQVPGTAPKLLIYGNTYRPSGVPDRFSGSKSGTSASLAITGLQAEDEADYYCQSYDNSLSGVVFGGGTKLTVL

SEQ ID NO: 14 - protein, 108 aa, Homo sapiens
QSALTQPASVSGSPGQSITISCTGTSSDVGGYNYVSWYQQHPGKAPKLMIYEVSNRPSGVSNRFSGSKSGNTASLTISGLQAEDEADYYCSSYTSSSVFGGGTKLTVL

SEQ ID NO: 15 - protein, 109 aa, Homo sapiens
QSALTQPASVSGSPGQSITISCTGTSSDVGRYNSVSWYQHHPGKAPKVMIYEVSNRPSGVSTRFSGSKSGNTASLTISGLQAEDEADYYCSSYTSSSVVFGGGTKLTVL

SEQ ID NO: 16 - protein, 109 aa, Homo sapiens
QSALTQPASVSGSPGQSITISCTGTSSDVGGYNSVSWYQQHPGKPPKLMIYEVSNRPSGVSIRFSGSKSGNTASLTISGLQAEDEADYFCSSYTSTSMVFGGGTKLTVL

SEQ ID NO: 17 - protein, 109 aa, Homo sapiens; identical to SEQ ID NO: 16

SEQ ID NO: 18 - protein, 109 aa, Homo sapiens
QSALTQPASVSGSPGQSITISCTGTSSDVGGYNSVSWYQQHPGKPPKLMIYEVSNRPSGVSNRFSGSKSGNTASLTISGLQAEDEADYFCSSYTSTSMVFGGGTKLAVL

SEQ ID NO: 19 - protein, 109 aa, Homo sapiens
QSALTQPASVSGSPGQSITISCTGTSSDVGGYNSVSWYQQYPGKPPKLKIYEVSNRPSGVSNRFSGSKSGNTASLTISGLQAEDEADYFCSSYTSTSMVFGGGTKLTVL

SEQ ID NO: 20 - protein, 109 aa, Homo sapiens
QSALTQPASVSGSPGQSITISCTGTSSDVGGYNSVSWYQQHPGKPPKLMIYEVSNRPSGVSNRFSGSKSGNTASLTISGLQAEDEADYFCSSYTSTSMVFGGGTKLTVL

SEQ ID NO: 21 - protein, 109 aa, Homo sapiens; identical to SEQ ID NO: 20

SEQ ID NO: 22 - protein, 109 aa, Homo sapiens
QSALTQPASVSGSPGQSITISCTGTNSDVGGYNSVSWYQQHPGKPPKLMIYEVSNRPSGISNRFSGSKSGNTASLTISGLQAEDEADYFCSSYTSTSMVFGGGTKLTVL

SEQ ID NO: 23 - protein, 109 aa, Homo sapiens
QSALTQPASVSGSPGQSITISCTGTSSDVGGYNSVSWYQQHPGKAPKLMIYEVSNRPSGVSNRFSGSKSGNTASLTISGLQAEDEADYYCNSYTSTSMVFGGGTKLTVL

SEQ ID NO: 24 - protein, 109 aa, Homo sapiens
QSALTQPASVSGSPGQSITISCTGTSSDVGAYNSVSWYQQHPGKAPKRMIYEVSNRPSGVSNRFSGSKSGNTASLTISGLQAEDEADYYCSSYTSTNMVFGGGTKLTVL

SEQ ID NO: 25 - protein, 108 aa, Homo sapiens; identical to SEQ ID NO: 14

SEQ ID NO: 26 - protein, 109 aa, Homo sapiens
QSALTQPASVSGSPGQSITISCTGTSSDVGGYNSVSWYQQHPGKAPKLMIYEVTNRPSGVSNRFSGSKSGNTASLTISGLQAEDEADYYCNSYTSTSMVFGGGTKLTVL

SEQ ID NO: 27 - protein, 108 aa, Homo sapiens
QSALTQPASVSGSPGQSITISCTGTSSDVGSYNLVSWYQQHPGKAPKLMIYEGSKRPSGVSNRFSGSKSGNTASLTISGLQAEDEADYYCCSYAGSSTFGGGTKLTVL

SEQ ID NO: 28 - protein, 110 aa, Homo sapiens
LSALTQPASVSGSPGQSITISCTGTSSDVGNYNLVSWYQQYSGKAPKLMIYEVSKRPSGVSNRFSGSKSGNTASLTISGLQAEDEADYYCCSYAGSSTLVFGGGTKLTVL

SEQ ID NO: 29 - protein, 108 aa, Homo sapiens
QSVLTQPPSASGTPGQRVTISCSGSSSNIGSNTVNWYQQLPGTAPKLLIYSNNQRPSGVPDRFSGSKSGTSASLAISGLQSEDEADYYCAAWDDSLNVFGGGTKLTVL

SEQ ID NO: 30 - protein, 109 aa, Homo sapiens
QSVLTQPPSASGTPGQRVTISCSGSSSNIGSKTVNWYQQVPGTAPKLLIYRNNQRPLGVPDRFSGSKSGTSASLAISGLQSEDEADYYCAAWDDSLNWVFGGGTKLTVL

SEQ ID NO: 31 - protein, 109 aa, Homo sapiens
QSVLTQPPSASGPPGQRVTISCSGSSSNIGSNTVNWYQQLPGTAPKLLIYSNNRRPSGVPDRFSGSKSGTSASLAISGLQSEDEADYYCAAWDDSLNWVFGGGTKLTVL

SEQ ID NO: 32 - protein, 110 aa, Homo sapiens
QSVLTQPPSASGTPGQRVTISCSGSSSNIGSNTVNWYQQLPGTAPKLLIYSNNQRPSGVPDRFSGSKSGTSASLAISGLQSEDEADYYCAVWDDSLNGWVFGGGTKLTVL

SEQ ID NO: 33 - protein, 109 aa, Homo sapiens
QSVLTQPPSASGTPGQRVTISCSGSSSNIGSKTVNWYQQFPGTAPKLLIYSNNRRPSGVPDRFSGSKSGTSASLAISGLQSEDEADYYCAAWDDSLNWVFGAGTKLTVL

SEQ ID NO: 34 - protein, 110 aa, Homo sapiens
QSVLTQPPSVSAAPGQKVTISCSGSSSNIGNNYVSWYQQLPGTAPKLLIYDNNKRPSGIPDRFSGSKSGTSATLGITGLQTGDEADYYCGTWDSSLSAYVFGTGTKVTVL

SEQ ID NO: 35 - protein, 110 aa, Homo sapiens
QSVLTQPPSVSAAPGQKVTISCSGSSSNIGNNFVSWYQQLPGTAPKLLIYDYNKRPSGIPDRFSGSKSGTSATLGITGLQTGDEADYYCGTWDSSLSAYVFGTGTRVTVL

SEQ ID NO: 36 - protein, 110 aa, Homo sapiens
QSVLTQPPSVSAAPGQKVTISCSGSSSNIGNNFVSWYQQLPGTAPKLLIYDYNKRPSGIPDRFSGSKSGTSATLGITGLQTGDEADYYCGTWDSSLSGYVFGTGTRVTVL

SEQ ID NO: 37 - protein, 110 aa, Homo sapiens
QSVLTQPPSVSAAPGQKVTISCSGSSSNIGNNFVSWYQQFPGTAPKLLIYDYNKRPSGIPDRFSGSKSGTSATLGITGLQTGDEADYYCGTWDSSLSSYVFGTGTRVTVL

SEQ ID NO: 38 - protein, 110 aa, Homo sapiens; identical to SEQ ID NO: 36

SEQ ID NO: 39 - protein, 110 aa, Homo sapiens
QSVLTQPPTVSAAPGQKVTISCSGSSSNIGNNFVSWYQQLPGTAPKLLIYDYNKRPSGIPDRFSGSKSGTSATLGITGLQTGDEADYYCGTWDSSLSGYVFGTGTRVTVL

SEQ ID NO: 40 - protein, 110 aa, Homo sapiens
QSVLTQPPSVSAAPGQKVTISCSGSSSNIGNNFVSWYQQLPGTAPKLLIYDSNKRPSGIPDRFSGSKSGTSATLDITGLQTGDEADYYCGTWDSSLSAYVFGTGTKVTVL

SEQ ID NO: 41 - protein, 110 aa, Homo sapiens
QSVLTQPPSVSAAPGQKVTISCSGSSSNIGNNYVSWYQQLPGTAPKLLIYDNNKRPSGIPDRFSGSKSGTSATLGITGLQTGDEADYYCGTWDSSLSAVVFGGGTKLTVL

SEQ ID NO: 42 - protein, 110 aa, Homo sapiens
QSVLTQPPSVSAAPGQKVTISCSGSNSNIGNNYVSWYQQLPGTAPKLLIYDNNKRPSGIPDRFSGSNSGTSATLGITGLQTGDEADYYCGTWDSSLSAVVFGGGTKLTVL

SEQ ID NO: 43 - protein, 107 aa, Homo sapiens
SYELTQPPSVSVSPGQTASITCSGDKLGDKYACWYQQKPGQSPVLVIYQDSKRPSGIPERFSGSNSGNTATLTISGTQAMDEADYYCQAWDSSTAVVFGGGTKLTVL

SEQ ID NO: 44 - protein, 106 aa, Homo sapiens
SYELTQPPSVSVSPGQTARITCSGDKLGDKYACWYQQKPGQSPVLVIYQNTKWPLGIPERFSGSKSGNTVTLTISGTQAMDEADYYCQAWDSSTVVFGGGTKLTVL

SEQ ID NO: 45 - protein, 116 aa, Homo sapiens
QPVLTQPPSASASLGASVTLTCTLSSGYSNYKVDWYQQRPGKGPRFVMRVGTGGIVGSKGDGIPDRFSVLGSGLNRYLTIKNIQEEDESDYHCGADHGSGSNFVVVFGGGTKLTVL

SEQ ID NO: 46 - protein, 116 aa, Homo sapiens
QPVLTQPLFASASLGASVTLTCTLSSGYSSYEVDWYQQRPGKGPRFVMRVDTGGIVGSKGEGIPDRFSVLGSGLNRYLTIKNIQEEDESDYHCGADHGSGTNFVVVFGGGTKLTVL

SEQ ID NO: 47 - protein, 114 aa, Homo sapiens
QVQLVQSGAEVKKPGASVKVSCKASGYTFTSYGISWVRQAPGQGLEWMGWISAYNGNTNYAQKLQGRVTMTTDTSTSTAYMELRSLRSDDTAVYYCARYGMDVWGQGTTVTVSS

SEQ ID NO: 48 - protein, 115 aa, Homo sapiens
QIQLVQSGAEVKKPGASVKVSCKASGYPLTSYGISWVRQAPGQGLEWMGWISAYNGNTNYAQKVQGSVTMTTDTSTSTVYMELRSLRSDDTAVYYCARGYGMDVWGQGTTVTVSS

SEQ ID NO: 49 - protein, 115 aa, Homo sapiens
QVQLVQSGAEVKKPGASVKVSCKASGYTLTSYGISWVRQAPGQGLEWMGWVSFYNGNTNYAQKLQGRGTMTTDPSTSTAYMELRSLRSDDTAVYYCARGYGMDVWGQGTTVTVSS

SEQ ID NO: 50 - protein, 115 aa, Homo sapiens; identical to SEQ ID NO: 49

SEQ ID NO: 51 - protein, 115 aa, Homo sapiens
QVQLVQSGAEVKKPGASVKVSCKASGYTLTSYGISWVRQAPGQGLEWMGWISFYNGNTNYAQKVQGRVTMTTDTSTSTVYMELRSLRSDDTAVYYCARGYGMDVWGQGTTVTVSS

SEQ ID NO: 52 - protein, 115 aa, Homo sapiens
QVQLVQSGAEVKRPGASVKVSCKASGYTLTSYGISWVRQAPGQGLEWMGWISVYNGNTNYAQKVQGRVTMTTDTSTSTVYMELRSLSSDDTAVYYCARGYGMDVWGQGTTVTVSS

SEQ ID NO: 53 - protein, 115 aa, Homo sapiens
QIQLVQSGAEVKKPGASVKVSCKASGYTLTSYGISWVRQAPGQGLEWMGWISFYNGNTNYAQKVQGRVTMTTDTSTSTVYMELRSLRSDDTAVYFCARGYGMDVWGQGTTVTVSS

SEQ ID NO: 54 - protein, 115 aa, Homo sapiens
QVQLVQSGAEVKKPGASLKVSCKASGYSLTSYGISWVRQAPGQGLEWMGWISAYNGNTNYAQKVQGRVTMTTDTSTSTVYMEVRSLRSDDTAVYYCARGYGMDVWGQGTTVTVSS

SEQ ID NO: 55 - protein, 115 aa, Homo sapiens
QVQLVQSGAEVKKPGASVKVSCKASGYPLTSYGISWVRQAPGQGLEWMGWISAYNGNTNYAQKVQGRVTMTTDTSTSTVYMELRSLRSDDTAVYYCARGYGMDVWGQGTTVTVSS

SEQ ID NO: 56 - protein, 115 aa, Homo sapiens
QVQLVQSGAEVKKPGASVKVSCKASGYALTSYGISWVRQAPGQGLEWMGWISAYNGNTNYAQKVQGRVTMTTDTSTSTVYMELRSLRSDDTAVYYCARGYGMDVWGQGTTVTVSS

SEQ ID NO: 57 - protein, 115 aa, Homo sapiens
QVQLVQSGAEVKKPGASVKVSCKASGYSFTSYGISWVRQAPGQGLEWMGWVSAYNGNTNYAQKFQGRVTMTTDTSTSTAYMELRSLRSDDTAVYYCARGYVMDVWGQGTTVTVSS

SEQ ID NO: 58 - protein, 115 aa, Homo sapiens
QVQLVQSGAEVKKPGASVKVSCKASGYTFPSYGISWVRQAPGQGLEWMGWISAYNGNTNYAEKLQGRVTMTTDTSTSTAYMEVRSLRSDDTAVFYCARGYVMDVWGQGTTVTVSS

SEQ ID NO: 59 - protein, 113 aa, Homo sapiens
QVQLVQSGAEVKKPGASVKVSCKASGYTFTSYGISWVRQAPGQGLEWMGWISAYNGNTNYAQKLQGRVTMTTDTSTSTAYMELRSLRSDDTAVYYCARGYDYWGQGTLVTVSS

SEQ ID NO: 60 - protein, 115 aa, Homo sapiens
QVQLVQSGAEVKKPGASVKVSCKASGYTFTSYGISWVRQAPGQGLEWMGWISTYNGNTNYAQKVQGRVTMTTDTSTSTAYMELRSLRSDDTAVYYCARGYTRDYWGQGTLVTVSS

SEQ ID NO: 61 - protein, 116 aa, Homo sapiens
EVQLVESGGGLVQPGGSLRLSCAASGFTFSSYWMSWVRQAPGKGLEWVANIKQDGSEKYYVDSVKGRFTISRDNAKNSLYLQMNSLRAEDTAVYYCARNWGAFDVWGQGTMVTVSS

SEQ ID NO: 62 - protein, 119 aa, Homo sapiens
EVQLVESGGGLVQPGGSLRLSCAASGFTFSRYWMSWVRQAPGKGLEWVANIKHDGSEKYYVDSVKGRFTISRDNAKNSLYLQMNSLRAEDTAVYYCARESNWGFAFDVWGHGTMVTVSS

SEQ ID NO: 63 - protein, 116 aa, Homo sapiens
EVQLVESGGGLVQPGGSLRLSCAASGFTFSSYWMSWVRQAPGKGLEWVANIKQDGSEKYYVDSVKGRFTISRDNAKNSLYLQMNSLRAEDTAVYYCARNWGAFDIWGQGTMVTVSS

SEQ ID NO: 64 - protein, 119 aa, Homo sapiens
EVQLVESGGGLVQPGGSLRLSCVVSGFTFSSYWMSWVRQAPGKGLEWVANIKQDGSEKYYVDSVKGRFTISRDNAKNSLYLQMNSLRAEDTAVYYCARESNWGFAFDIWGQGTMVTVSS

SEQ ID NO: 65 - protein, 119 aa, Homo sapiens
EVQLVESGGGLVQPGGSLRLSCAASGLTFSNFWMSWVRQAPGKGLEWVANIKQDGSEKYYVDSVKGRFTISRDNAKNSLYLQMNSLRAEDTAVYSCTRESNWGFAFDIWGQGTMVTVSS

SEQ ID NO: 66 - protein, 123 aa, Homo sapiens
EVQLVESGGGLVKPGGSLRLSCAASGFTFSSYSMNWVRQAPGKGLEWVSSISSSSSYIYYADSVKGRFTISRDNAKNSLYLQMNSLRAEDTAVYYCARDYDFWSGYYTAFDVWGQGTMVTVSS

SEQ ID NO: 67 - protein, 123 aa, Homo sapiens
EVQLVESGGGLVKPGGSLRLSCAASGFTFSSYSMNWVRQAPGKGLEWVSSISSSSSYISYADSVKGRFTISRDNAKNSLYLQMNSLRAEDTAVYFCARDYDFWSAYYDAFDVWGQGTMVTVSS

SEQ ID NO: 68 - protein, 112 aa, Homo sapiens
EVQLLESGGGLVQPGGSLRLSCAASGFTFSSYAMSWVRQAPGKGLEWVSAISGSGGSTYYADSVKGRFTISRDNSKNTLYLQMNSLRAEDTAVYYCAKFDYWGQGTLVTVSS

SEQ ID NO: 69 - protein, 117 aa, Homo sapiens
EVQLLESGGGLVQPGGSLRLSCAASGFTFSSYAMSWVRQAPGKGLEWVSTISGSGGRTYYADSVKGRFTISRDNSKNTLYLQMNSLRAEDTAVYYCAKEVGSPFDYWGQGTLVTVSS

SEQ ID NO: 70 - protein, 117 aa, Homo sapiens
EVQLLESGGGLVQPGGSLRLSCAASGFTFSSYAMSWVRQAPGKGLEWVSAISGSGGSTYYADSVKGRFTISRDNSKNTLYLQMNSLRAEDTAVYYCAKVLMVYADYWGQGTLVTVSS

SEQ ID NO: 71 - protein, 121 aa, Homo sapiens
EVQLLESGGGLVQPGGSLRLSCAASGFTFSSYAMNWVRQAPGKGLEWVSTISGSGDNTYYADSVKGRFTISRDNSKNTLYLQMNSLRAEDTAVYYCAKKFVLMVYAMLDYWGQGTLVTVSS

SEQ ID NO: 72 - protein, 121 aa, Homo sapiens
EVQLLESGGGLVQPGGSLRLSCAASGFTFSSYAMNWVRQAPGKGLEWVSTISGSGGNTYYADSVKGRFTISRDNSKNTLYLQMNSLRAEDTAVYYCAKKFVLMVYAMLDYWGQGTLVTVSS

SEQ ID NO: 73 - protein, 116 aa, Homo sapiens
QVQLVESGGGVVQPGRSLRLSCAASGFTFSSYGMHWVRQAPGKGLEWVAVIWYDGSNKYYADSVKGRFTISRDNSKNTLYLQMNSLRAEDTAVYYCARYYYGMDVWGQGTTVTVSS

SEQ ID NO: 74 - protein, 123 aa, Homo sapiens
QVQLVESGGGVVQPGRSLRLSCAASGFTFSSYGMHWVRQAPGKGLEWVAVIWYDGSDKYYADSVKGRFTISRDNSKNTLYLQMNSLRAEDTAVYYCARETGPLKLYYYGMDVWGQGTTVTVSS

SEQ ID NO: 75 - protein, 116 aa, Homo sapiens
QVQLVESGGGVVQPGRSLRLSCAASGFTFSSYGMHWVRQAPGKGLEWVAVIWYDGSNKYYADSVKGRFTISRDNSKNTLYLQMNSLRAEDTAVYYCARIAAGMDVWGQGTTVTVSS

SEQ ID NO: 76 - protein, 122 aa, Homo sapiens
QVHLVESGGGVVQPGRSLRLSCAASGFTFNSFGMHWVRQAPGKGLEWVALIWSDGSDKYYADSVKGRFTISRDNSKNTLYLQMNSLRAEDTAVYYCARAIAALYYYYGMDVWGQGTTVTVSS

SEQ ID NO: 77 - protein, 122 aa, Homo sapiens
QVQLVESGGGVVQPGRSLRLSCAASGFTFSSFGMHWVRQAPGKGLEWVALIWNDGSNKYYADSVKGRFTISRDNSKNTLYLQMNSLRAEDTAVYYCARAIAALYYYYGMDVWGHGTTVTVSS

SEQ ID NO: 78 - protein, 122 aa, Homo sapiens
QVQLVESGGGVVQPGRSLRLSCAASGFTFSSFGMHWVRQAPGKGLEWVALIWNDGSNKYYADSVKGRFTISRDNSKNTLYLQMNSLRAEDTAVYYCARAIAALYYYYGMDVWGQGTTVTVSS

SEQ ID NO: 79 - protein, 122 aa, Homo sapiens
QVHLVESGGGVVQPGRSLRLSCAASGFTFNSFGMHWVRQAPGKGLEWVALIWSDGSDEYYADSVKGRFTISRDNSKNTLYLQMNSLRAEDTAVYYCARAIAALYYYYGMDVWGQGTTVTVSS

SEQ ID NO: 80 - protein, 122 aa, Homo sapiens; identical to SEQ ID NO: 78

SEQ ID NO: 81 - protein, 122 aa, Homo sapiens
QVQLVESGGGVVQPGRSLRLSCAASGFTFSSYGMHWVRQAPGKGLEWVAIIWYDGSNKYYADSVKGRFTISRDNSKNTLYLQMNSLRAEDTAVYYCARRGGLAARPGGMDVWGQGTTVTVSS

SEQ ID NO: 82 - protein, 122 aa, Homo sapiens
QVQLVESGGGVVQPGRSLRLSCAASGFTFSSYGMHWVRQAPGKGLEWVAVIWYDGSNKYYADSVKGRFTISRDNSKNTLYLQMNSLRAEDTAVYYCARGIAVAYYYYGMDVWGQGTTVTVSS

SEQ ID NO: 83 - protein, 122 aa, Homo sapiens
QVQLVESGGGVVQPGRSLRLSCAASGFTFRSYGMHWVRQAPGKGLEWVALIWHDGSNTYYVDSVKGRFTISRDNSKNTLYLQMNSLRAEDTAVYYCARGIAVAYYYYGMDVWGQGTTVTVSS

SEQ ID NO: 84 - protein, 117 aa, Homo sapiens
QVQLQESGPGLVKPSQTLSLTCTVSGGSISSGGYYWSWIRQHPGKGLEWIGYIYYSGSTYYNPSLKSRVTISVDTSKNQFSLKLSSVTAADTAVYYCARYYYGMDVWGQGTTVTVSS

SEQ ID NO: 85 - protein, 122 aa, Homo sapiens
QVQLQESGPGLVKPSQTLSLTCTVSGGSISSSDYYWSWIRQHPGKGLEWIGYIYYSGSTYYNPSLKSRITISVDTSKNLFSLKLSSVTAADTAVYYCARGGVTTYYYAMDVWGQGTTVTVSS

SEQ ID NO: 86 - protein, 120 aa, Homo sapiens
QVQLQESGPGLVKPSQTLSLTCTVSGGSISSGGYYWSWIRQHPGKGLEWIGYIYYSGSTYYNPSLKSRVTISVDTSKNQFSLKLSSVTAADTAVYYCAREDTAMVYFDYWGQGTLVTVSS

SEQ ID NO: 87 - protein, 121 aa, Homo sapiens
QVQLQESGPGLVKPSQTLSLTCTVSGGSISSGGYYWSWIRQHPGKGLEWIGYIYNSGSTYYNPSLKSRVTISVDTSKNQFSLKLSSVTAADTAVYYCAREDTAMVPYFDYWGQGTLVTVSS

SEQ ID NO: 88 - protein, 115 aa, Homo sapiens
QVQLQQWGAGLLKPSETLSLTCAVYGGSFSGYYWSWIRQPPGKGLEWIGEINHSGSTNYNPSLKSRVTISVDTSKNQFSLKLSSVTAADTAVYYCARGQLVFDYWGQGTLVTVSS

SEQ ID NO: 89 - protein, 116 aa, Homo sapiens
QVQLQQWGAGLLKPSETLSLTCAVYGGSFSAYYWNWIRQPPGKGLEWIGEINHSGRTDYNPSLKSRVTISVDTSKKQFSLKLNSVTAADTAVYYCARGQLVPFDYWGQGTLVTVSS

SEQ ID NO: 90 - protein, 115 aa, Homo sapiens
QVQLQQSGPGLVKPSQTLSLTCAISGDSVSSNSAAWNWIRQSPSRGLEWLGRTYYRSKWYNDYAVSVKSRITINPDTSKNQFSLQLNSVTPEDTAVYYCARFDYWGQGTLVTVSS

SEQ ID NO: 91 - protein, 121 aa, Homo sapiens
QVQLQQSGPGLVKPSQTLSLTCAISGDSVSSNSAAWNWIRQSPSRGLEWLGRTYYRSKWYKNYSVSVKSRITINPDTSKNQFSLQLNSVTPGDTAVYYCARGGPTAAFDYWGQGTLVTVSS

SEQ ID NO: 92 - DNA, 345 bp, Homo sapiens
  source 1..345: mol_type = unassigned DNA
cagattcagctggtgcagtctggagctgaggtgaagaagcctggggcctcagtgaaggtctcctgcaaggcttctggttaccccttgaccagctatggtatcagctgggtgcgacaggcccctggacaagggcttgagtggatgggatggatcagcgcttacaatggtaacacaaactatgcacagaaggtccagggcagcgtcaccatgaccacagacacatccacgagcacagtctacatggagctgaggagcctgagatctgacgacacggccgtgtattactgtgcgagaggctacggtatggacgtctggggccaagggaccacggtcaccgtctcctct

SEQ ID NO: 93 - DNA, 327 bp, Homo sapiens
  source 1..327: mol_type = unassigned DNA
cagtctgccctgactcagcctgcctccgtgtctgggtctcctggacagtcgatcaccatctcctgcactggaaccagcagtgacgttggtggttataactctgtctcctggtaccaacagtacccaggcaaaccccccaaactcaagatttatgaggtcagtaatcggccctcaggggtttctaatcgcttctctggctccaagtctggcaacacggcctccctgaccatctctgggctccaggctgaggacgaggctgattatttctgcagctcatatacaagcaccagcatggtcttcggcggagggaccaagctgaccgtccta

SEQ ID NO: 94 - DNA, 345 bp, Homo sapiens
  source 1..345: mol_type = unassigned DNA
caggttcagctggtgcagtctggagctgaggtgaagaagcctggggcctcagtgaaggtctcctgcaaggcttctggttacaccttaaccagctatggtatcagctgggtgcgacaggcccctggacaagggcttgagtggatgggatgggtcagtttttataatggtaacacaaactatgcacagaagctccagggcagaggcaccatgaccacagacccatccacgagcacagcctacatggagctgaggagcctgagatctgacgacacggccgtgtattactgtgcgagaggctacggtatggacgtctggggccaagggaccacggtcaccgtctcctct

SEQ ID NO: 95 - DNA, 327 bp, Homo sapiens
  source 1..327: mol_type = unassigned DNA
cagtctgccctgactcagcctgcctccgtgtctgggtctcctggacagtcgatcaccatctcctgcactggaaccagcagtgacgttggtggttataactctgtctcctggtaccaacagcacccaggcaaagcccccaaactcatgatttatgaggtcagtaatcggccctcaggggtttctaatcgcttctctggctccaagtctggcaacacggcctccctgaccatctctgggctccaggctgaggacgaggctgattattactgcaattcatatacaagcaccagcatggtattcggcggagggaccaagctgaccgtccta

SEQ ID NO: 96 - DNA, 345 bp, Homo sapiens
  source 1..345: mol_type = unassigned DNA
caggttcagctggtgcagtctggagctgaagtgaagaagcctggggcctcagtgaaggtctcctgcaaggcttctggttacaccttgaccagctatggtatcagctgggtgcgacaggcccctggacaagggcttgagtggatgggatggatcagcttttacaatggtaacacaaactatgcacagaaggtccagggcagagtcaccatgaccacagacacatccacgagcacagtctacatggagctgaggagcctgagatctgacgacacggccgtgtattactgtgcgagaggctacggtatggacgtctggggccaagggaccacggtcaccgtctcctct

SEQ ID NO: 97 - DNA, 327 bp, Homo sapiens
  source 1..327: mol_type = unassigned DNA
cagtctgccctgactcagcctgcctccgtgtctgggtctcctggacagtcgatcaccatctcctgcactggaaccagcagtgacgttggtggttataactctgtctcctggtaccaacagcacccaggcaaaccccccaaactcatgatttatgaggtcagtaatcggccctcaggggtttctattcgcttctctggctccaagtctggcaacacggcctccctgaccatctctgggctccaggctgaggacgaggctgattatttctgcagctcatatacaagcaccagcatggtcttcggcggagggaccaagctgaccgtccta

SEQ ID NO: 98 - DNA, 345 bp, Homo sapiens
  source 1..345: mol_type = unassigned DNA
cagattcagctggtgcagtctggagctgaggtgaagaagcctggggcctcagtgaaggtctcctgcaaggcttctggttacaccttgaccagctatggtatcagctgggtgcgacaggcccctggacaagggcttgagtggatgggatggatcagcttttacaatggtaacacaaactatgcacagaaggtccagggcagagtcaccatgaccacagacacatccacgagcacagtctacatggagctgaggagcctgagatctgacgacacggccgtgtatttctgtgcgagaggttacggtatggacgtctggggccaagggaccacggtcaccgtctcctca

SEQ ID NO: 99 - DNA, 327 bp, Homo sapiens
  source 1..327: mol_type = unassigned DNA
cagtctgccctgactcagcctgcctccgtgtctgggtctcctggacagtcgatcaccatctcctgcactggaaccagcagtgacgttggtggttataactctgtctcgtggtaccaacagcacccaggcaaaccccccaaactcatgatttatgaggtcagtaatcggccctcaggggtttctaatcgcttctctggctccaagtctggcaacacggcctccctgaccatctctgggctccaggctgaggacgaggctgattatttctgcagctcatatacaagcaccagcatggtcttcggcggagggaccaagctggccgtccta

SEQ ID NO: 100 - DNA, 345 bp, Homo sapiens
  source 1..345: mol_type = unassigned DNA
caggttcagctggtgcagtctggagctgaggtgaagaagcctggggcctcagtgaaggtctcctgcaaggcttctggttacaccttaaccagctatggtatcagctgggtgcgacaggcccctggacaagggcttgagtggatgggatgggtcagtttttataatggtaacacaaactatgcacagaagctccagggcagaggcaccatgaccacagacccatccacgagcacagcctacatggagctgaggagcctgagatctgacgacacggccgtgtattactgtgcgagaggctacggtatggacgtctggggccaagggaccacggtcaccgtctcctca

SEQ ID NO: 101 - DNA, 327 bp, Homo sapiens
  source 1..327: mol_type = unassigned DNA
cagtctgccctgactcagcctgcctccgtgtctgggtctcctggacagtcgatcaccatctcctgcactggaaccagcagtgacgttggtggttataactctgtctcctggtaccaacagcacccaggcaaagcccccaaactcatgatttatgaggtcactaatcggccctcaggggtttctaatcgcttctctggctccaagtctggcaacacggcctccctgaccatctctgggctccaggctgaggacgaggctgattattactgcaactcatatacaagcaccagcatggtgttcggcggagggaccaagctgaccgtccta

SEQ ID NO: 102 - DNA, 363 bp, Homo sapiens
  source 1..363: mol_type = unassigned DNA
caggtgcagctgcaggagtcgggcccaggactggtgaagccttcacagaccctgtccctcacctgcactgtctctggtggctccatcagcagtggtggttactactggagctggatccgccagcacccagggaagggcctggagtggattgggtacatatataacagtgggagcacctactacaacccgtccctcaagagtcgagttaccatatcagtagacacgtctaagaaccagttctccctgaagctgagctctgtgactgccgcggacacggccgtgtattactgtgcgagagaggatacagctatggttccttactttgactactggggccagggaaccctggtcaccgtctcctca

SEQ ID NO: 103 - DNA, 333 bp, Homo sapiens
  source 1..333: mol_type = unassigned DNA
cagtctgtactgacgcagccgccctcagtgtctggggccccagggcagagggtcaccatctcctgcactgggagcagctccaacatcggggcacattatgatgtgcactggtaccagcaggttccaggaacagcccccaaactcctcatctatggtaacacctatcggccctcaggggtccctgaccgattctctggctccaagtctggcacctcagcctccctggccatcactgggctccaggctgaggatgaggctgattattactgccagtcctatgacaacagcctgagtggtgtggtattcggcggagggaccaagctgaccgtccta

SEQ ID NO: 104 - DNA, 366 bp, Homo sapiens
  source 1..366: mol_type = unassigned DNA
caggtgcacctggtggagtctgggggaggcgtggtccagcctgggaggtccctgagactctcctgtgcagcgtctggattcaccttcaacagctttggcatgcactgggtccgccaggctccaggcaaggggctggagtgggtggcacttatctggtctgatggaagtgatgaatactatgcagactccgtgaagggccgattcaccatctccagagacaattccaagaacacgctgtatctgcaaatgaacagcctgagagccgaggacacggctgtgtattactgtgcgagagccatagcagccctctactactactacggtatggacgtctggggccaagggaccacggtcaccgtctcctca

SEQ ID NO: 105 - DNA, 330 bp, Homo sapiens
  source 1..330: mol_type = unassigned DNA
cagtctgtgttgacgcagccgccctcagtgtctgcggccccaggacagaaggtcaccatctcctgctctggaagcagctccaacattgggaataattttgtatcctggtaccagcagctcccaggaacagcccccaaactcctcatttatgactataataagcgaccctcagggattcctgaccgattctctggctccaagtctggcacgtcagccaccctgggcatcaccggactccagactggggacgaggccgattattactgcggaacatgggatagcagcctgagtgcttatgtcttcggaactgggaccagggtcaccgtccta

SEQ ID NO: 106 - DNA, 366 bp, Homo sapiens
  source 1..366: mol_type = unassigned DNA
caggtgcagctggtggagtctgggggaggcgtggtccagcctgggaggtccctgagactctcctgtgcagcgtctggattcaccttcagcagctttggcatgcactgggtccgccaggctccaggcaaggggctggagtgggtggcacttatatggaatgatggaagtaataaatactatgcagactccgtgaagggccgattcaccatctccagagacaattccaagaacacgctgtatctgcaaatgaacagcctgagagccgaggacacggctgtgtattactgtgcgagagccatagcagccctctactactactacggtatggacgtctggggccaagggaccacggtcaccgtctcctca

SEQ ID NO: 107 - DNA, 330 bp, Homo sapiens
  source 1..330: mol_type = unassigned DNA
cagtctgtgttgacgcagccgccctcagtgtctgcggccccaggacagaaggtcaccatctcctgctctggaagcagctccaacattgggaataattttgtatcctggtaccagcagctcccaggaacagcccccaaactcctcatttatgactataataagcgaccctcagggattcctgaccgattctctggctccaagtctggcacgtcagccaccctgggcatcaccggactccagactggggacgaggccgattattactgcggaacatgggatagcagtctgagtggttatgtcttcggaactgggaccagggtcaccgtccta

SEQ ID NO: 108 - DNA, 366 bp, Homo sapiens
  source 1..366: mol_type = unassigned DNA
caggtgcacctggtggagtctgggggaggcgtggtccagcctgggaggtccctgagactctcctgtgcagcgtctggattcaccttcaacagctttggcatgcactgggtccgccaggctccaggcaaggggctggagtgggtggcacttatatggtctgatggaagtgataaatactatgcagactccgtgaagggccgattcaccatctccagagacaattccaagaacacgctgtatctgcaaatgaacagcctgagagccgaggacacggctgtgtattactgtgcgagagccatagcagccctctactactactacggtatggacgtctggggccaagggaccacggtcaccgtctcctca

SEQ ID NO: 109 - DNA, 330 bp, Homo sapiens
  source 1..330: mol_type = unassigned DNA
cagtctgtgttgacgcagccgccctcagtgtctgcggccccaggacagaaggtcaccatctcctgctctggaagcagttccaacattgggaataattttgtatcctggtaccagcagttcccaggaacagcccccaaactcctcatttatgactataataagcgaccctcagggattcctgaccgattctctggctccaagtctggcacgtcagccaccctgggcatcaccggactccagactggggacgaggccgattattactgcggaacatgggatagcagcctgagttcttatgtcttcggaactgggaccagggtcaccgtccta

SEQ ID NO: 110 - DNA, 366 bp, Homo sapiens
  source 1..366: mol_type = unassigned DNA
caggtgcagctggtggagtctgggggaggcgtggtccagcctgggaggtccctgagactctcctgtgcagcgtctggattcaccttcagcagctttggcatgcactgggtccgccaggctccaggcaaggggctggagtgggtggcacttatatggaatgatggaagtaataaatactatgcagactccgtgaagggccgattcaccatctccagagacaattccaagaacacgctgtatctgcaaatgaacagcctgagagccgaggacacggctgtgtattactgtgcgagagccatagcagccctctactactactacggtatggacgtctggggccacgggaccacggtcaccgtctcctca

SEQ ID NO: 111 - DNA, 330 bp, Homo sapiens
  source 1..330: mol_type = unassigned DNA
cagtctgtgttgacgcagccgccctcagtgtctgcggccccaggacagaaggtcaccatctcctgctctggaagcagctccaacattgggaataattttgtatcctggtaccagcagctcccaggaacagcccccaaactcctcatttatgactataataagcgaccctcagggattcctgaccgattctctggctccaagtctggcacgtcagccaccctgggcatcaccggactccagactggggacgaggccgattattactgcggaacatgggatagcagcctgagtggttatgtcttcggaactgggaccagggtcaccgtccta

SEQ ID NO: 112 - DNA, 366 bp, Homo sapiens; identical to SEQ ID NO: 106
  source 1..366: mol_type = unassigned DNA

SEQ ID NO: 113 - DNA, 330 bp, Homo sapiens
  source 1..330: mol_type = unassigned DNA
cagtctgtgttgacgcagccgcccacagtgtctgcggccccaggacagaaggtcaccatctcctgctctggaagcagctccaacattgggaataattttgtatcctggtaccagcagctcccaggaacagcccccaaactcctcatttatgactataataagcgaccctcagggattcctgaccgattctctggctccaagtctggcacgtcagccaccctgggcatcaccggactccagactggggacgaggccgattactactgcggaacatgggatagcagcctgagtggttatgtcttcggaactgggaccagggtcaccgtccta

SEQ ID NO: 114 - DNA, 366 bp, Homo sapiens
  source 1..366: mol_type = unassigned DNA
caggtgcagctggtggagtctgggggaggcgtggtccagcctgggaggtccctgagactctcctgtgcagcgtctggattcaccttcaggagctatggcatgcactgggtccgccaggctccaggcaaggggctggagtgggtggcacttatatggcatgatggaagtaatacatactatgtagactccgtgaagggccgattcaccatctccagagacaattccaagaacacgctgtatctgcaaatgaacagcctgagagccgaggacacggctgtgtattactgtgcgagaggtatagcagtggcttactactactacggtatggacgtctggggccaagggaccacggtcaccgtctcctca

SEQ ID NO: 115 - DNA, 330 bp, Homo sapiens
  source 1..330: mol_type = unassigned DNA
cagtctgtgttgacgcagccgccctcagtgtctgcggccccaggacagaaggtcaccatctcctgctctggaagcagctccaacattgggaataattttgtatcctggtaccagcagctcccaggaacagcccccaaactcctcatttatgacagtaataagcgaccctcagggattcctgaccgattctctggctccaagtctggcacgtcagccaccctggacatcaccggactccagactggggacgaggccgattattactgcggaacatgggatagcagcctgagtgcttatgttttcggaactgggaccaaggtcaccgtccta

SEQ ID NO: 116 - DNA, 363 bp, Homo sapiens
  source 1..363: mol_type = unassigned DNA
gaggtgcagctgttggagtctgggggaggcttggtacagcctggggggtccctgagactctcctgtgcagcctctggattcacctttagcagctatgccatgaactgggtccgccaggctccagggaaggggctggagtgggtctcaactattagtggtagtggtgataacacatactacgcagactccgtgaagggccggttcaccatctccagagacaattccaagaacacgctgtatctgcaaatgaacagcctgagagccgaggacacggccgtatattactgtgcgaaaaagtttgtactaatggtgtatgctatgcttgactactggggccagggaaccctggtcaccgtctcctca

SEQ ID NO: 117 - DNA, 321 bp, Homo sapiens
  source 1..321: mol_type = unassigned DNA
gacatcctgatgacccagtctccatcctccctgtctgcatctgttggagacagagtcaccatcacttgccgggcaagtcagagcattagcagttatttaaattggtatcagcagaaaccagggaaagcccctaaggtcctgatctatgctgcctccagtttgcaaagtggggtcccatcaaggttcagtggcagtggatctgggacagatttcactctcaccatcaacagtctgcaacctgaagattttgcaacttactactgtcaacagagttacagttcccccatcaccttcggccaagggacacgactggagattaaa

SEQ ID NO: 118 - DNA, 363 bp, Homo sapiens
  source 1..363: mol_type = unassigned DNA
gaggtgcagctgttggagtctgggggaggcttggtacagccgggggggtccctgagactctcctgtgcagcctctggattcacctttagcagctatgccatgaactgggtccgccaggctccagggaaggggctggagtgggtctcaactattagtggtagtggtggtaacacatactacgcagactccgtgaagggccggttcaccatctccagagacaattccaagaacacgctgtatctgcaaatgaacagcctgagagccgaggacacggccgtatattactgtgcgaaaaagtttgtactaatggtgtatgctatgcttgactactggggccagggaaccctggtcaccgtctcctca

SEQ ID NO: 119 - DNA, 321 bp, Homo sapiens
  source 1..321: mol_type = unassigned DNA
gacatccagatgacccagtctccatcctccctatctgcatctgtaggagacagagtcaccatcacttgccgggcaagtcagagcattagcatctatttaaattggtatcagcagaagccagggaaagccccttacctcctgatctatgctgcagccagtttgcaaagtggggtcccatcaaggttcagtggcagtggatctgggacagatttcactctcaccatcagcagtctgcaacctgaagattttgcaacttactactgtcaacagagttacagtgcccccatcaccttcggccaagggacacgactggagattaaa

SEQ ID NO: 120 - DNA, 345 bp, Homo sapiens
  source 1..345: mol_type = unassigned DNA
caggttcagctggtgcagtctggagctgaggtgaagaagcctggggcctcactgaaggtctcctgcaaggcttctggttacagtttgaccagctatggtatcagctgggtgcgacaggcccctggacaagggcttgagtggatgggatggatcagcgcttacaatggtaacacaaactatgcacagaaggtccagggcagagtcaccatgaccacagacacatccacgagcacagtctacatggaggtgaggagtctgagatctgacgacacggccgtgtattactgtgcgagaggctacggtatggacgtctggggccaagggaccacggtcaccgtctcctca

SEQ ID NO: 121 - DNA, 327 bp, Homo sapiens
  source 1..327: mol_type = unassigned DNA
cagtctgccctgactcagcctgcctccgtgtctgggtctcctggacagtcgatcaccatctcctgcactggaaccagcagtgacgttggtggttataactctgtctcctggtaccaacagcacccaggcaaaccccccaaactcatgatttatgaggtcagtaatcggccctcaggggtttctaatcgcttctctggctccaagtctggcaatacggcctccctgaccatctctgggctccaggctgaggacgaggctgattatttctgcagctcatatacaagcaccagcatggtcttcggcggagggaccaagctgaccgtccta

SEQ ID NO: 122 - DNA, 345 bp, Homo sapiens
  source 1..345: mol_type = unassigned DNA
caggttcagctggtgcagtctggagctgaggtgaagaggcctggggcctcagtgaaggtctcctgcaaggcttctggttacaccttgaccagctatggtatcagctgggtgcgacaggcccctggacaagggcttgagtggatgggatggatcagcgtttacaatggtaacacaaactatgcacagaaggtccagggcagagtcaccatgaccacagacacatccacgagcacagtctacatggagctgaggagcctgagctctgacgacacggccgtgtattactgtgcgagaggctacggtatggacgtctggggccaagggaccacggtcaccgtctcctca

SEQ ID NO: 123 - DNA, 327 bp, Homo sapiens; identical to SEQ ID NO: 97
  source 1..327: mol_type = unassigned DNA

SEQ ID NO: 124 - DNA, 345 bp, Homo sapiens
  source 1..345: mol_type = unassigned DNA
caggttcagctggtgcagtctggagctgaggtgaagaagcctggggcctcagtgaaggtctcctgcaaggcttctggttaccccttgaccagctatggtatcagctgggtgcgacaggcccctggacaagggcttgagtggatgggatggatcagcgcttacaatggtaacacaaactatgcacagaaggtccagggcagagtcaccatgaccacagacacatccacgagcacagtctacatggagttgaggagcctgagatctgacgacacggccgtgtattactgtgcgagaggctacggtatggacgtctggggccaagggaccacggtcaccgtctcctca

SEQ ID NO: 125 - DNA, 327 bp, Homo sapiens; identical to SEQ ID NO: 121
  source 1..327: mol_type = unassigned DNA

SEQ ID NO: 126 - DNA, 345 bp, Homo sapiens
  source 1..345: mol_type = unassigned DNA
caggttcagttggtgcagtctggagctgaggtgaagaagcctggggcctcagtgaaggtctcctgcaaggcttctggttacgccttgaccagctatggtatcagctgggtgcgacaggcccctggacaagggcttgagtggatgggatggatcagcgcttacaatggtaacacaaactatgcacagaaggtccagggcagagtcaccatgaccacagacacatccacgagcacagtctacatggagctgaggagcctgagatctgacgacacggccgtgtattactgtgcgagaggctacggtatggacgtctggggccaagggaccacggtcaccgtctcctca

SEQ ID NO: 127 - DNA, 327 bp, Homo sapiens
  source 1..327: mol_type = unassigned DNA
cagtctgccctgactcagcctgcctccgtgtctgggtctcctggacagtcgatcaccatctcctgcactggaaccaacagtgacgttggtggttataactctgtctcctggtaccaacagcacccaggcaaaccccccaaactcatgatttatgaggtcagtaatcggccctcagggatttctaatcgcttctctggctccaagtctggcaacacggcctccctgaccatctctgggctccaggctgaggacgaggctgattatttctgcagctcatatacaagcaccagcatggtcttcggcggagggaccaagctgaccgtccta

SEQ ID NO: 128 - DNA, 345 bp, Homo sapiens
  source 1..345: mol_type = unassigned DNA
caggttcagctggtgcagtctggagctgaggtgaagaagcctggggcctcagtgaaggtctcctgcaaggcttctggttacagctttaccagctatggtatcagctgggtgcgacaggcccctggacaagggcttgagtggatgggatgggtcagcgcttacaatggtaacacaaactatgcacagaagttccagggcagagtcaccatgaccacagacacatccacgagcacagcctacatggaactgaggagcctgagatctgacgacacggccgtgtattactgtgcgagaggctacgttatggacgtctggggccaagggaccacggtcaccgtctcctca

SEQ ID NO: 129 - DNA, 327 bp, Homo sapiens
  source 1..327: mol_type = unassigned DNA
cagtctgccctgactcagcctgcctccgtttctgggtctcctggacagtcgatcaccatctcctgcactggaaccagcagtgacgttggtgcttataactctgtctcctggtaccaacagcacccaggcaaagcccccaaacgcatgatttatgaggtcagtaatcggccctcaggggtttctaatcgcttctctggctccaagtctggcaacacggcctccctgaccatctctgggctccaggctgaggacgaggctgattattactgcagctcatatacaagcaccaacatggtattcggcggagggaccaagctgaccgtccta

SEQ ID NO: 130 - DNA, 363 bp, Homo sapiens
  source 1..363: mol_type = unassigned DNA
caggtacagttgcagcagtcaggtccaggactggtgaagccctcgcagaccctctcactcacctgtgccatctccggggacagtgtctctagcaacagtgctgcttggaactggatcaggcagtccccatcgagaggccttgagtggctgggaaggacatactacaggtccaagtggtataaaaattattcagtatctgtgaaaagtcgaataaccatcaacccagacacatccaagaaccagttctctctgcaactgaactctgtgactcccggggacacggctgtgtattactgtgcaagaggggggccaactgctgcttttgactactggggccagggaaccctggtcaccgtctcctca

SEQ ID NO: 131 - DNA, 330 bp, Homo sapiens
  source 1..330: mol_type = unassigned DNA
ctttctgccctgactcagcctgcctccgtgtctgggtctcctggacagtcgatcaccatctcctgcactggaaccagcagtgatgttgggaattataaccttgtctcctggtaccaacagtattcaggcaaagcccccaaactcatgatttatgaggtcagtaagcggccctcaggggtttctaatcgcttctctggctccaagtctggcaacacggcctccctgacaatctctgggctccaggctgaggacgaggctgattattactgctgctcatatgcaggtagtagcactttggttttcggcggagggaccaagctgaccgtccta

SEQ ID NO: 132 - DNA, 357 bp, Homo sapiens
  source 1..357: mol_type = unassigned DNA
gaggtgcagttggtggagtctgggggaggcttggtccagcctggggggtccctgagactctcctgtgtagtctctggattcacctttagtagctattggatgagctgggtccgccaggctccagggaaggggctggagtgggtggccaacataaagcaagatggaagtgagaaatactatgtggactctgtgaagggccgattcaccatctccagagacaacgccaagaactcactgtatctgcaaatgaacagcctgagagccgaggacacggctgtatattactgtgcgagagagtcaaactggggatttgcttttgatatctggggccaagggacaatggtcaccgtctcttca

SEQ ID NO: 133 - DNA, 327 bp, Homo sapiens
  source 1..327: mol_type = unassigned DNA
cagtctgtgctgactcagccaccctcagcgtctgggacccccgggcagagggtcaccatctcttgttctggaagcagctccaacatcggaagtaagactgtaaactggtaccaacaggtcccaggaacggcccccaaactcctcatctataggaataatcagcggcccttaggggtccctgaccgattctctggctccaagtctggcacctcagcctccctggccatcagtgggctccagtctgaggatgaggctgattattattgtgcagcatgggatgacagcctgaattgggtgttcggcggagggaccaagctgaccgtccta

SEQ ID NO: 134 - DNA, 357 bp, Homo sapiens
  source 1..357: mol_type = unassigned DNA
gaggtgcagctggtggagtctgggggaggcttggtccagcctggggggtccctgagactctcctgtgcagcctctggattcacctttagtcgctattggatgagctgggtccgccaggctccagggaaggggctggagtgggtggccaacataaagcatgatggaagtgagaaatactatgtggactctgtgaagggccgattcaccatttccagagacaacgccaagaactcactgtatctgcaaatgaacagcctgagagccgaggacacggctgtgtattactgtgcgagagagtcaaactggggatttgcttttgatgtctggggccacgggacaatggtcaccgtctcttca

SEQ ID NO: 135 - DNA, 327 bp, Homo sapiens
  source 1..327: mol_type = unassigned DNA
cagtctgtgctgactcagccaccctcagcgtctgggccccccggacagagggtcaccatctcttgttctggaagcagctccaacatcggaagtaatactgtaaactggtaccagcagctcccaggaacggcccccaaactcctcatctatagtaataatcggcggccctcaggggtccctgaccgattctctggctccaagtctggcacctcagcctccctggccatcagtgggctccagtctgaggatgaggctgattattactgtgcagcatgggatgacagcctgaattgggtgttcggcggagggaccaagctgaccgtccta

SEQ ID NO: 136 - DNA, 351 bp, Homo sapiens
  source 1..351: mol_type = unassigned DNA
gaggtgcagctgttggagtctgggggaggcttggtacagcctggggggtccctgagactctcctgtgcagcctctggattcacctttagcagctatgccatgagctgggtccgccaggctccagggaaggggctggagtgggtctcaactattagtggtagtggtggtaggacatattacgcagactccgtgaagggccggttcaccatctccagagacaattccaagaacacgctgtatctgcaaatgaacagcctgagagccgaggacacggccgtatattactgtgcgaaagaagttggcagtccctttgactactggggccagggaaccctggtcaccgtctcctca

SEQ ID NO: 137 - DNA, 330 bp, Homo sapiens
  source 1..330: mol_type = unassigned DNA
cagtctgtgttgacgcagccgccctcagtgtctgcggccccaggacagaaggtcaccatctcctgctctggaagcaactccaacattgggaataattatgtatcctggtaccagcagctcccaggaacagcccccaaactcctcatttatgacaataataagcgaccctcagggattcctgaccgattctctggctccaactctggcacgtcagccaccctgggcatcaccggactccagactggggacgaggccgattattactgcggaacatgggatagcagcctgagtgctgtggtattcggcggagggaccaagctgaccgtccta

SEQ ID NO: 138 - DNA, 366 bp, Homo sapiens
  source 1..366: mol_type = unassigned DNA
caggtgcagctggtggagtctgggggaggcgtggtccagcctgggaggtccctgagactctcctgtgcagcgtctggattcaccttcagtagctatggcatgcactgggtccgccaggctccaggcaaggggctggagtgggtggcaattatatggtatgatggaagtaataaatactatgcagactccgtgaagggccgattcaccatctccagagacaattccaagaacacactgtatcttcaaatgaacagcctgagagccgaggacacggctgtgtattactgtgcgaggagggggggtctggcagctcgtccgggcggtatggacgtctggggccaagggaccacggtcaccgtctcctca

SEQ ID NO: 139 - DNA, 318 bp, Homo sapiens
  source 1..318: mol_type = unassigned DNA
tcctatgagctgactcagccaccctcagtgtctgtgtccccaggacagacagccagaatcacctgctctggagataaattgggggataaatatgcttgctggtatcagcagaaaccaggccagtcccctgtgctggtcatctatcaaaataccaagtggcccttagggatccctgagcgattctctggctccaagtctgggaacacagtcactctgaccatcagcgggacccaggctatggatgaggctgactattactgtcaggcgtgggacagcagcactgtggtattcggcggagggaccaagctgaccgtccta

SEQ ID NO: 140 - DNA, 366 bp, Homo sapiens
  source 1..366: mol_type = unassigned DNA
caggtgcagctgcaggagtcgggcccaggactggtgaagccttcacagaccctgtccctcacctgcactgtctctggtggctccatcagcagtagtgattactactggagctggatccgccagcacccagggaagggcctggagtggattgggtacatctattacagtgggagcacctactacaacccgtccctcaagagtcgaattaccatatcagtagacacgtctaagaacctgttctccctgaagttgagctctgtgactgccgcggacacggccgtgtattactgtgcgagagggggggtgactacgtactactacgctatggacgtctggggccaagggaccacggtcaccgtctcctca

SEQ ID NO: 141 - DNA, 321 bp, Homo sapiens
  source 1..321: mol_type = unassigned DNA
gacatacagatgacccagtctccatcctccctgtctgcatctgtaggagacagagtcaccatcacttgccgggcaagtcagcgcattagcaactatttaagttggtatctgcagaaaccagggattgcccctaagctcctgatctatgctgcatccagtttgcagagtggggtcccatcaaggttcagtggcagtggatctgggacagatttcactctcaccatcagcagtctgcaatctgaagattttgcaacttactactgtcaacagagttacagtaccccgctcattttcggcggagggaccaaggtggagatcaaa

SEQ ID NO: 142 - DNA, 369 bp, Homo sapiens
  source 1..369: mol_type = unassigned DNA
caggtgcagctggtggagtctgggggaggcgtggtccagcctgggaggtccctgagactctcctgtgcagcgtctggattcaccttcagtagctatggcatgcactgggtccgccaggctccaggcaaggggctggagtgggtggcagttatatggtatgatggaagtgataaatactatgcagactccgtgaagggccgattcaccatctccagagacaattccaagaacacgctgtatctgcaaatgaacagcctgagagccgaggacacggctgtgtattactgtgcgagagagactggtcccttgaaactctactactacggtatggacgtctggggccaagggaccacggtcaccgtctcctca

SEQ ID NO: 143 - DNA, 336 bp, Homo sapiens
  source 1..336: mol_type = unassigned DNA
gatattgtgatgactcagtctccactctccctgtccgtcacccctggagagccgccctccatctcctgcaggtctagtcagagcctcctgcatagtaatggatacaactttttgaattggtacctgcagaagccagggcagtctccacaactcctgatctatttgggttctcatcgggcctccggggtccctgacaggttcagtggcagtggatcaggcacagattttacactggaaatcagcagagtggaggctgaggatgttggggtttattactgcatgcaagttctacaaactccattcactttcggccctgggaccaaagtggatatcaaa

SEQ ID NO: 144 - DNA, 357 bp, Homo sapiens
  source 1..357: mol_type = unassigned DNA
gaggtgcagctggtggagtctgggggaggcttggtccagcctggggggtccctgagactctcctgtgcagcctctggactcacctttagtaacttttggatgagctgggtccgccaggctccagggaaggggctggagtgggtggccaacataaagcaagatggaagtgagaaatactatgtggactctgtgaagggccgattcaccatctccagagacaacgccaagaattcactgtatctgcaaatgaacagcctgagagccgaggacacggctgtgtattcctgtacgagagagtcaaactggggatttgcttttgatatctggggccaagggacaatggtcaccgtctcttca

SEQ ID NO: 145 - DNA, 327 bp, Homo sapiens
  source 1..327: mol_type = unassigned DNA
cagtctgtgctgactcagccaccctcagcgtctgggacccccgggcagagggtcaccatctcttgttctggaagcagctccaacatcggaagtaaaactgtaaactggtaccagcagttcccaggaacggcccccaaactcctcatctatagtaataatcggcggccctcaggggtccctgaccgattctctggctccaagtctggcacctcagcctccctggccatcagtgggctccagtctgaggatgaggctgattattactgtgcagcatgggatgacagcctgaattgggtgttcggcgcagggaccaagctgaccgtccta

SEQ ID NO: 146 - DNA, 345 bp, Homo sapiens
  source 1..345: mol_type = unassigned DNA
caggttcagctggtgcagtctggagctgaggtgaagaagcctggggcctcagtgaaggtctcctgcaaggcttctggttacacctttaccagctatggtatcagctgggtgcgacaggcccctggacaagggcttgagtggatgggatggatcagcacttacaatggtaacacaaactatgcacagaaggtccagggcagagtcaccatgaccacagacacatccacgagcacagcctacatggagctgaggagcctgagatctgacgacacggccgtttattactgtgcgagagggtatactcgggactactggggccagggaaccctggtcaccgtctcctca

SEQ ID NO: 147 - DNA, 348 bp, Homo sapiens
  source 1..348: mol_type = unassigned DNA
cagcctgtgctgactcagccactttttgcatcagcctccctgggagcctcggtcacactcacctgcaccctgagcagcggctacagtagttatgaagtggactggtatcagcagagaccagggaagggcccccggtttgtcatgcgagtggacactggtgggattgtgggatccaagggggaaggcatccctgatcgcttctcagttttgggctcaggcctgaatcggtatctgaccatcaagaacatccaggaagaggatgagagtgactaccactgtggggcagaccatggcagtgggaccaacttcgtggtggtattcggcggagggaccaagctgaccgtccta

SEQ ID NO: 148 - DNA, 348 bp, Homo sapiens
  source 1..348: mol_type = unassigned DNA
caggtgcagctacagcagtggggcgcaggactgttgaagccttcggagaccctgtccctcacctgcgctgtctatggtgggtccttcagtgcgtactactggaactggatccgccagcccccagggaaggggctggagtggattggggaaatcaatcatagtggaagaaccgactacaacccgtccctcaagagtcgagtcaccatatcagtagacacgtccaagaagcagttctccctgaagctgaactctgtgaccgccgcggacacggctgtgtattactgtgcgagagggcagctcgtcccctttgactactggggccagggaaccctggtcaccgtctcttca

SEQ ID NO: 149 - DNA, 330 bp, Homo sapiens
  source 1..330: mol_type = unassigned DNA
cagtctgtgctgactcagccaccctcagcgtctgggacccccgggcagagggtcaccatctcttgttctggaagcagctccaacatcggaagtaatactgtaaattggtatcagcaactcccaggaacggcccccaaactcctcatctatagtaataatcagcggccctcaggggtccctgaccgattctctggctccaagtctggcacctcagcctccctggccatcagtgggctccagtctgaggatgaggctgattattactgtgcagtatgggatgacagcctgaatggttgggtgttcggcggagggaccaagctgaccgtccta

SEQ ID NO: 150 - DNA, 345 bp, Homo sapiens
  source 1..345: mol_type = unassigned DNA
caggttcagctggtgcagtctggagctgaggtgaagaagcctggggcctcagtgaaggtctcctgcaaggcttctggttacacctttcccagctatggtatcagctgggtgcgacaggcccctggacaagggcttgagtggatgggatggatcagcgcttacaatggtaacacaaactatgcagagaagctccagggcagagtcaccatgaccacagacacatccacgagcacagcctacatggaggtgaggagcctgagatctgacgacacggccgtgttttactgtgcgagaggctacgttatggacgtctggggccaagggaccacggtcaccgtctcctct

SEQ ID NO: 151 - DNA, 327 bp, Homo sapiens
  source 1..327: mol_type = unassigned DNA
cagtctgccctgactcagcctgcctccgtgtctgggtctcctggacagtcgatcaccatctcctgcactggaaccagcagtgacgttggtcgttataattctgtctcctggtaccaacaccacccaggcaaagcccccaaagtcatgatttatgaggtcagtaatcggccctcaggggtttctactcgcttctctggctccaagtctggcaacacggcctccctgaccatctctgggctccaggctgaggacgaggctgattattactgcagctcatatacaagcagcagcgttgtattcggcggagggaccaaactgaccgtccta

SEQ ID NO: 152 - DNA, 369 bp, Homo sapiens
  source 1..369: mol_type = unassigned DNA
gaggtgcagctggtggagtctgggggaggcctggtcaagcctggggggtccctgagactctcctgtgcagcctctggattcaccttcagtagctatagcatgaactgggtccgccaggctccagggaaggggctggagtgggtctcatccattagtagtagtagtagttacatttcctacgcagactcagtgaagggccgattcaccatctccagagacaacgccaagaactcactgtatctgcaaatgaacagcctgagagccgaggacacggctgtgtatttctgtgcgagagattacgatttttggagtgcttactatgatgcttttgatgtctggggccaagggacaatggtcaccgtctcttca

SEQ ID NO: 153 - DNA, 333 bp, Homo sapiens
  source 1..333: mol_type = unassigned DNA
cagtctgtgctgacgcagccgccctcagtgtctggggccccagggcagagggtcaccatctcctgcactgggagcagctccaacatcggggcaggttatgatgtacactggtaccagcagcttccaggaacagcccccaaactcctcatctctggtaacagcaatcggccctcaggggtccctgaccgattctctggctccaagtctggcacctcagcctccctggccatcactgggctccaggctgaggatgaggctgattattactgccagtcctatgacagcagcctgagtggttcggtattcggcggagggaccaagctgaccgtccta

SEQ ID NO: 154 - protein, 326 aa, Homo sapiens
ASTKGPSVFPLAPCSRSTSESTAALGCLVKDYFPEPVTVSWNSGALTSGVHTFPAVLQSSGLYSLSSVVTVPSSNFGTQTYTCNVDHKPSNTKVDKTVERKCCVECPPCPAPPVAGPSVFLFPPKPKDTLMISRTPEVTCVVVDVSHEDPEVQFNWYVDGVEVHNAKTKPREEQFNSTFRVVSVLTVVHQDWLNGKEYKCKVSNKGLPAPIEKTISKTKGQPREPQVYTLPPSREEMTKNQVSLTCLVKGFYPSDIAVEWESNGQPENNYKTTPPMLDSDGSFFLYSKLTVDKSRWQQGNVFSCSVMHEALHNHYTQKSLSLSPGK

SEQ ID NO: 155 - protein, 327 aa, Homo sapiens
ASTKGPSVFPLAPCSRSTSESTAALGCLVKDYFPEPVTVSWNSGALTSGVHTFPAVLQSSGLYSLSSVVTVPSSSLGTKTYTCNVDHKPSNTKVDKRVESKYGPPCPSCPAPEFLGGPSVFLFPPKPKDTLMISRTPEVTCVVVDVSQEDPEVQFNWYVDGVEVHNAKTKPREEQFNSTYRVVSVLTVLHQDWLNGKEYKCKVSNKGLPSSIEKTISKAKGQPREPQVYTLPPSQEEMTKNQVSLTCLVKGFYPSDIAVEWESNGQPENNYKTTPPVLDSDGSFFLYSRLTVDKSRWQEGNVFSCSVMHEALHNHYTQKSLSLSLGK

SEQ ID NO: 156 - protein, 105 aa, Homo sapiens
QPKAAPSVTLFPPSSEELQANKATLVCLISDFYPGAVTVAWKADSSPVKAGVETTTPSKQSNNKYAASSYLSLTPEQWKSHRSYSCQVTHEGSTVEKTVAPTECS

SEQ ID NO: 157 - protein, 106 aa, Homo sapiens
TVAAPSVFIFPPSDEQLKSGTASVVCLLNNFYPREAKVQWKVDNALQSGNSQESVTEQDSKDSTYSLSSTLTLSKADYEKHKVYACEVTHQGLSSPVTKSFNRGEC

SEQ ID NO: 158 - protein, 14 aa, Homo sapiens
TGTSSDVGGYNSVS

SEQ ID NO: 159 - protein, 14 aa, Homo sapiens
TGTNSDVGGYNSVS

SEQ ID NO: 160 - protein, 14 aa, Homo sapiens
TGTSSDVGAYNSVS

SEQ ID NO: 161 - protein, 14 aa, Homo sapiens
TGTSSDVGRYNSVS

SEQ ID NO: 162 - protein, 7 aa, Homo sapiens
EVSNRPS

SEQ ID NO: 163 - protein, 7 aa, Homo sapiens
EVTNRPS

SEQ ID NO: 164 - protein, 9 aa, Homo sapiens
SSYTSTSMV

SEQ ID NO: 165 - protein, 9 aa, Homo sapiens
NSYTSTSMV

SEQ ID NO: 166 - protein, 9 aa, Homo sapiens
SSYTSTNMV

SEQ ID NO: 167 - protein, 9 aa, Homo sapiens
SSYTSSSVV

SEQ ID NO: 168 - protein, 10 aa, Homo sapiens
GYPLTSYGIS

SEQ ID NO: 169 - protein, 10 aa, Homo sapiens
GYSLTSYGIS

SEQ ID NO: 170 - protein, 10 aa, Homo sapiens
GYALTSYGIS

SEQ ID NO: 171 - protein, 10 aa, Homo sapiens
GYTLTSYGIS

SEQ ID NO: 172 - protein, 10 aa, Homo sapiens
GYSFTSYGIS

SEQ ID NO: 173 - protein, 10 aa, Homo sapiens
GYTFPSYGIS

SEQ ID NO: 174 - protein, 17 aa, Homo sapiens
WISAYNGNTNYAQKVQG

SEQ ID NO: 175 - protein, 17 aa, Homo sapiens
WVSFYNGNTNYAQKLQG

SEQ ID NO: 176 - protein, 17 aa, Homo sapiens
WISFYNGNTNYAQKVQG

SEQ ID NO: 177 - protein, 17 aa, Homo sapiens
WISVYNGNTNYAQKVQG

SEQ ID NO: 178 - protein, 17 aa, Homo sapiens
WVSAYNGNTNYAQKFQG

SEQ ID NO: 179 - protein, 17 aa, Homo sapiens
WISAYNGNTNYAEKLQG

SEQ ID NO: 180 - protein, 6 aa, Homo sapiens
GYGMDV

SEQ ID NO: 181 - protein, 6 aa, Homo sapiens
GYVMDV

SEQ ID NO: 182 - protein, 13 aa, Homo sapiens
SGSSSNIGNNFVS

SEQ ID NO: 183 - protein, 7 aa, Homo sapiens
DYNKRPS

SEQ ID NO: 184 - protein, 7 aa, Homo sapiens
DSNKRPS

SEQ ID NO: 185 - protein, 11 aa, Homo sapiens
GTWDSSLSGYV

SEQ ID NO: 186 - protein, 11 aa, Homo sapiens
GTWDSSLSAYV

SEQ ID NO: 187 - protein, 11 aa, Homo sapiens
GTWDSSLSSYV

SEQ ID NO: 188 - protein, 10 aa, Homo sapiens
GFTFSSFGMH

SEQ ID NO: 189 - protein, 10 aa, Homo sapiens
GFTFNSFGMH

SEQ ID NO: 190 - protein, 10 aa, Homo sapiens
GFTFRSYGMH

SEQ ID NO: 191 - protein, 17 aa, Homo sapiens
LIWNDGSNKYYADSVKG

SEQ ID NO: 192 - protein, 17 aa, Homo sapiens
LIWSDGSDEYYADSVKG

SEQ ID NO: 193 - protein, 17 aa, Homo sapiens
LIWSDGSDKYYADSVKG

SEQ ID NO: 194 - protein, 17 aa, Homo sapiens
LIWHDGSNTYYVDSVKG

SEQ ID NO: 195 - protein, 13 aa, Homo sapiens
AIAALYYYYGMDV

SEQ ID NO: 196 - protein, 13 aa, Homo sapiens
GIAVAYYYYGMDV

SEQ ID NO: 197 - protein, 13 aa, Homo sapiens
SGSSSNIGSNTVN

SEQ ID NO: 198 - protein, 13 aa, Homo sapiens
SGSSSNIGSKTVN

SEQ ID NO: 199 - protein, 7 aa, Homo sapiens
SNNRRPS

SEQ ID NO: 200 - protein, 7 aa, Homo sapiens
RNNQRPL

SEQ ID NO: 201 - protein, 10 aa, Homo sapiens
AAWDDSLNWV

SEQ ID NO: 202 - protein, 10 aa, Homo sapiens
GFTFSRYWMS

SEQ ID NO: 203 - protein, 10 aa, Homo sapiens
GLTFSNFWMS

SEQ ID NO: 204 - protein, 10 aa, Homo sapiens
GFTFSSYWMS

SEQ ID NO: 205 - protein, 17 aa, Homo sapiens
NIKHDGSEKYYVDSVKG

SEQ ID NO: 206 - protein, 17 aa, Homo sapiens
NIKQDGSEKYYVDSVKG

SEQ ID NO: 207 - protein, 10 aa, Homo sapiens
ESNWGFAFDV

SEQ ID NO: 208 - protein, 10 aa, Homo sapiens
ESNWGFAFDI

SEQ ID NO: 209 - protein, 11 aa, Homo sapiens
RASQSISSYLN

SEQ ID NO: 210 - protein, 11 aa, Homo sapiens
RASQSISIYLN

SEQ ID NO: 211 - protein, 7 aa, Homo sapiens
AASSLQS

SEQ ID NO: 212 - protein, 7 aa, Homo sapiens
AAASLQS

SEQ ID NO: 213 - protein, 9 aa, Homo sapiens
QQSYSSPIT

SEQ ID NO: 214 - protein, 9 aa, Homo sapiens
QQSYSAPIT

SEQ ID NO: 215 - protein, 10 aa, Homo sapiens
GFTFSSYAMN

SEQ ID NO: 216 - protein, 17 aa, Homo sapiens
TISGSGDNTYYADSVKG

SEQ ID NO: 217 - protein, 17 aa, Homo sapiens
TISGSGGNTYYADSVKG

SEQ ID NO: 218 - protein, 12 aa, Homo sapiens
KFVLMVYAMLDY

SEQ ID NO: 219 - protein, 11 aa, Homo sapiens
RASQRISNYLS

SEQ ID NO: 220 - protein, 16 aa, Homo sapiens
RSSQSLLHSNGYNFLN

SEQ ID NO: 221 - protein, 14 aa, Homo sapiens
TGTSSDVGNYNLVS

SEQ ID NO: 222 - protein, 14 aa, Homo sapiens
TGSSSNIGAGYDVH

SEQ ID NO: 223 - protein, 14 aa, Homo sapiens
TGSSSNIGAHYDVH

SEQ ID NO: 224 - protein, 13 aa, Homo sapiens
SGSNSNIGNNYVS

SEQ ID NO: 225 - protein, 11 aa, Homo sapiens
SGDKLGDKYAC

SEQ ID NO: 226 - protein, 12 aa, Homo sapiens
TLSSGYSSYEVD

SEQ ID NO: 227 - protein, 7 aa, Homo sapiens
LGSHRAS

SEQ ID NO: 228 - protein, 7 aa, Homo sapiens
EVSKRPS

SEQ ID NO: 229 - protein, 7 aa, Homo sapiens
GNSNRPS

SEQ ID NO: 230 - protein, 7 aa, Homo sapiens
GNTYRPS

SEQ ID NO: 231 - protein, 7 aa, Homo sapiens
SNNQRPS

SEQ ID NO: 232 - protein, 7 aa, Homo sapiens
DNNKRPS

SEQ ID NO: 233 - protein, 7 aa, Homo sapiens
QNTKWPL

SEQ ID NO: 234 - protein, 7 aa, Homo sapiens
VDTGGIV

SEQ ID NO: 235 - protein, 9 aa, Homo sapiens
QQSYSTPLI

SEQ ID NO: 236 - protein, 9 aa, Homo sapiens
MQVLQTPFT

SEQ ID NO: 237 - protein, 10 aa, Homo sapiens
CSYAGSSTLV

SEQ ID NO: 238 - protein, 11 aa, Homo sapiens
QSYDSSLSGSV

SEQ ID NO: 239 - protein, 11 aa, Homo sapiens
QSYDNSLSGVV

SEQ ID NO: 240 - protein, 11 aa, Homo sapiens
AVWDDSLNGWV

SEQ ID NO: 241 - protein, 11 aa, Homo sapiens
GTWDSSLSAVV

SEQ ID NO: 242 - protein, 9 aa, Homo sapiens
QAWDSSTVV

SEQ ID NO: 243 - protein, 18 aa, Homo sapiens
SDYHCGADHGSGTNFVVV

SEQ ID NO: 244 - protein, 10 aa, Homo sapiens
GYTFTSYGIS

SEQ ID NO: 245 - protein, 10 aa, Homo sapiens
GFTFSSYAMS

SEQ ID NO: 246 - protein, 10 aa, Homo sapiens
GFTFSSYGMH

SEQ ID NO: 247 - protein, 10 aa, Homo sapiens
GFTFSSYSMN

SEQ ID NO: 248 - protein, 12 aa, Homo sapiens
GGSISSGGYYWS

SEQ ID NO: 249 - protein, 12 aa, Homo sapiens
GGSISSSDYYWS

SEQ ID NO: 250 - protein, 10 aa, Homo sapiens
GGSFSAYYWN

SEQ ID NO: 251 - protein, 12 aa, Homo sapiens
GDSVSSNSAAWN

SEQ ID NO: 252 - protein, 17 aa, Homo sapiens
WISTYNGNTNYAQKVQG

SEQ ID NO: 253 - protein, 17 aa, Homo sapiens
TISGSGGRTYYADSVKG

SEQ ID NO: 254 - protein, 17 aa, Homo sapiens
VIWYDGSDKYYADSVKG

SEQ ID NO: 255 - protein, 17 aa, Homo sapiens
IIWYDGSNKYYADSVKG

SEQ ID NO: 256 - protein, 17 aa, Homo sapiens
SISSSSSYISYADSVKG

SEQ ID NO: 257 - protein, 16 aa, Homo sapiens
YIYNSGSTYYNPSLKS

SEQ ID NO: 258 - protein, 16 aa, Homo sapiens
YIYYSGSTYYNPSLKS

SEQ ID NO: 259 - protein, 16 aa, Homo sapiens
EINHSGRTDYNPSLKS

SEQ ID NO: 260 - protein, 18 aa, Homo sapiens
RTYYRSKWYKNYSVSVKS

SEQ ID NO: 261 - protein, 6 aa, Homo sapiens
GYTRDY

SEQ ID NO: 262 - protein, 8 aa, Homo sapiens
EVGSPFDY

SEQ ID NO: 263 - protein, 14 aa, Homo sapiens
ETGPLKLYYYGMDV

SEQ ID NO: 264 - protein, 13 aa, Homo sapiens
RGGLAARPGGMDV

SEQ ID NO: 265 - protein, 14 aa, Homo sapiens
DYDFWSAYYDAFDV

SEQ ID NO: 266 - protein, 11 aa, Homo sapiens
EDTAMVPYFDY

SEQ ID NO: 267 - protein, 12 aa, Homo sapiens
GGVTTYYYAMDV

SEQ ID NO: 268 - protein, 8 aa, Homo sapiens
GQLVPFDY

SEQ ID NO: 269 - protein, 9 aa, Homo sapiens
GGPTAAFDY

SEQ ID NO: 270 - protein, 109 aa, Homo sapiens
QSALTQPASVSGSPGQSITISCTGTSSDVGGYNSVSWYQQHPGKAPKLMIYEVSNRPSGVFNRFSGSKSGNTASLTISGLQAEDEADYYCNSYTSTSMVFGGGTKLTVL

SEQ ID NO: 271 - protein, 109 aa, Homo sapiens
QSALTQPASVFGSPGQSITISCTGTSSDVGAYNSVSWYQQHPGKAPKRMIYEVSNRPSGVSNRFSGSKSGNTASLTISGLQAEDEADYYCSSYTSTNMVFGGGTKLTVL

SEQ ID NO: 272 - protein, 109 aa, Homo sapiens; identical to SEQ ID NO: 31

SEQ ID NO: 273 - protein, 109 aa, Homo sapiens
QSVLTQPPSASGPPGQRVTIFCSGSSSNIGSNTVNWYQQLPGTAPKLLIYSNNRRPSGVPDRFSGSKSGTSASLAISGLQSEDEADYYCAAWDDSLNWVFGGGTKLTVL

SEQ ID NO: 274 - protein, 106 aa, Homo sapiens
SYELTQPPSVSVSPGQTASITCSGDKLGDKYACWYQQKPGQSPVLVIYQDSKRPSGIPERFSGSNSGNTATLTISGTQAMDEADYYCQAWDSSTVVFGGGTKLTVL

SEQ ID NO: 275 - protein, 106 aa, Homo sapiens; identical to SEQ ID NO: 44

SEQ ID NO: 276 - protein, 107 aa, Homo sapiens; identical to SEQ ID NO: 43

SEQ ID NO: 277 - protein, 107 aa, Homo sapiens
SYELIQPPSVSVSPGQTASITCSGDKLGDKYACWYQRKPGQSPILVIYQDTKRPSGIPERFSGSNSGNTATLTISGTQAMDEADYYCQAWDSSTAVVFGGGTKLTVL

SEQ ID NO: 278 - protein, 120 aa, Homo sapiens
QVQLQESGPGLVKPSETLSLTCTVSGGSISTYYWSWIRQPPGKGLEWIGYIYYSGSTNYNPSLKSRVTISVDTSKNQFSLKLSSVTAADTAVYYCARGSYSSGWFEFDYWGQGTLVTVSS

SEQ ID NO: 279 - protein, 12 aa, Homo sapiens
TLSSGYSSYEVD

SEQ ID NO: 280 - protein, 12 aa, Homo sapiens
VDTGGIVGSKGE

SEQ ID NO: 281 - protein, 13 aa, Homo sapiens
GADHGSGTNFVVV

SEQ ID NO: 282 - protein, 22 aa, Homo sapiens
QPVLTQPLFASASLGASVTLTC

SEQ ID NO: 283 - protein, 15 aa, Homo sapiens
WYQQRPGKGPRFVMR

SEQ ID NO: 284 - protein, 32 aa, Homo sapiens
GIPDRFSVLGSGLNRYLTIKNIQEEDESDYHC

SEQ ID NO: 285 - protein, 10 aa, Homo sapiens
FGGGTKLTVL

SEQ ID NO: 286 - protein, 108 aa, Homo sapiens
QSALTQPASVSGSPGQSITISCTGTSSDVGRYNSVSWYQHHPGKAPKVMIYEVSNRPSGVSTRFSGSKSGNTASLTISGLQAEDEADYYCSSYTSSSVVFGGGTKLTV

SEQ ID NO: 287 - protein, 108 aa, Homo sapiens
QSALTQPASVSGSPGQSITISCTGTSSDVGGYNSVSWYQQHPGKPPKLMIYEVSNRPSGVSIRFSGSKSGNTASLTISGLQAEDEADYFCSSYTSTSMVFGGGTKLTV

SEQ ID NO: 288 - protein, 108 aa, Homo sapiens
QSALTQPASVSGSPGQSITISCTGTNSDVGGYNSVSWYQQHPGKPPKLMIYEVSNRPSGISNRFSGSKSGNTASLTISGLQAEDEADYFCSSYTSTSMVFGGGTKLTV

SEQ ID NO: 289 - protein, 122 aa, Homo sapiens
QVHLVESGGGVVQPGRSLRLSCAASGFTFSSFGMHWVRQAPGKGLEWVALIWNDGSNKYYADSVKGRFTISRDNSKNTLYLQMNSLRAEDTAVYYCARAIAALYYYYGMDVWGHGTTVTVSS

SEQ ID NO: 290 - protein, 122 aa, Homo sapiens
QVQLVESGGGVVQPGRSLRLSCAASGFTFSSYGMHWVRQAPGKGLECVAIIWYDGSNKYYADSVKGRFTISRDNSKNTLYLQMNSLRAEDTAVYYCARRGGLAARPGGMDVWGQGTTVTVSS

SEQ ID NO: 291 - protein, 121 aa, Homo sapiens
QVQLVESGGGVVQPGRSLRLSCAASGFTFSSFGMHWVRQAPGKGLEWVALIWNDGSNKYYADSVKGRFTISRDNSKNTLYLQMNSLRAEDTAVYYCARAIAALYYYYGMDVWGQGTTVTVS

SEQ ID NO: 292 - protein, 119 aa, Homo sapiens
QVQLVESGGGVVQPGRSLRLSCAASGFTFSSYGMHWVRQAPGKGLEWVAIIWYDGSNKYYADSVKGRFTISRDNSKNTLYLQMNSLRAEDTAVYYCARRGGLPGGMDVWGQGTTVTVSS

SEQ ID NO: 293 - DNA, 327 bp, Homo sapiens
  source 1..327: mol_type = unassigned DNA
cagtctgccctgactcagcctgcctccgtgtctgggtctcctggacagtcgatcaccatctcctgcactggaaccagcagtgacgttggtggttataactctgtctcctggtaccaacagcacccaggcaaagcccccaaactcatgatttatgaggtcagtaatcggccctcaggggtttctaatcgcttctctggctccaagtctggcaacacggcctccctgaccatctctgggctccaggctgaggacgaggctgattattactgcaactcatatacaagcaccagcatggtattcggcggagggaccaagctgaccgtccta

SEQ ID NO: 294 - DNA, 327 bp, Homo sapiens
  source 1..327: mol_type = unassigned DNA
cagtctgccctgactcagcctgcctccgtgtctgggtctcctggacagtcgatcaccatctcctgcactggaaccagcagtgacgttggtggttataactctgtctcctggtaccaacagcacccaggcaaaccccccaaactcatgatttatgaggtcagtaatcggccctcaggggtttctaatcgcttctctggctccaagtctggcaacacggcctccctgaccatctctgggctccaggctgaggacgaggctgattatttctgcagctcatatacaagcaccagcatggtcttcggcggagggaccaagctgaccgtccta

SEQ ID NO: 295 - DNA, 318 bp, Homo sapiens
  source 1..318: mol_type = unassigned DNA
tcctatgagctgactcagccaccctcagtgtccgtgtccccaggacagacagccagaatcacctgctctggagataaattgggggataaatatgcttgctggtatcagcagaagccaggccagtcccctgtgctggtcatctatcaaaataccaagtggcccttagggatccctgagcgattctctggctccaagtctgggaacacagtcactctgaccatcagcgggacccaggctatggatgaggctgactattactgtcaggcgtgggacagcagcactgtggtattcggcggagggaccaagctgaccgtccta

SEQ ID NO: 296 - DNA, 327 bp, Homo sapiens; identical to SEQ ID NO: 95
  source 1..327: mol_type = unassigned DNA

SEQ ID NO: 297 - protein, 215 aa, Homo sapiens
ESALTQPASVSGSPGQSITISCTGTSSDVGGYNSVSWYQQHPGKAPKLMIYEVSNRPSGVSNRFSGSKSGNTASLTISGLQAEDEADYYCNSYTSTSMVFGGGTKLTVLGQPKAAPSVTLFPPSSEELQANKATLVCLISDFYPGAVTVAWKADSSPVKAGVETTTPSKQSNNKYAASSYLSLTPEQWKSHRSYSCQVTHEGSTVEKTVAPTECS

SEQ ID NO: 298 - protein, 230 aa, Homo sapiens
EVQLVQSGAEVKKPGASVKVSCKASGYTLTSYGISWVRQAPGQGLEWMGWVSFYNGNTNYAQKLQGRGTMTTDPSTSTAYMELRSLRSDDTAVYYCARGYGMDVWGQGTTVTVSSASTKGPSVFPLAPSSKSTSGGTAALGCLVKDYFPEPVTVSWNSGALTSGVHTFPAVLQSSGLYSLSSVVTVPSSSLGTQTYICNVNHKPSNTKVDKKVEPKSCAADEVDHHHHHH

SEQ ID NO: 299 - protein, 217 aa, Homo sapiens
ESVLTQPPSVSGAPGQRVTISCTGSSSNIGAGYDVHWYQQLPGTAPKLLISGNSNRPSGVPDRFSGSKSGTSASLAITGLQAEDEADYYCQSYDSSLSGSVFGGGTKLTVLGQPKAAPSVTLFPPSSEELQANKATLVCLISDFYPGAVTVAWKADSSPVKAGVETTTPSKQSNNKYAASSYLSLTPEQWKSHRSYSCQVTHEGSTVEKTVAPTECS

SEQ ID NO: 300 - protein, 238 aa, Homo sapiens
EVQLVESGGGLVKPGGSLRLSCAASGFTFSSYSMNWVRQAPGKGLEWVSSISSSSSYISYADSVKGRFTISRDNAKNSLYLQMNSLRAEDTAVYFCARDYDFWSAYYDAFDVWGQGTMVTVSSASTKGPSVFPLAPSSKSTSGGTAALGCLVKDYFPEPVTVSWNSGALTSGVHTFPAVLQSSGLYSLSSVVTVPSSSLGTQTYICNVNHKPSNTKVDKKVEPKSCAADEVDHHHHHH

SEQ ID NO: 301 - protein, 218 aa, Homo sapiens
ALQSVLTQPPSASGTPGQRVTISCSGSSSNIGSNTVNWYQQLPGTAPKLLIYSNNQRPSGVPDRFSGSKSGTSASLAISGLQSEDEADYYCAVWDDSLNGWVFGGGTKLTVLGQPKAAPSVTLFPPSSEELQANKATLVCLISDFYPGAVTVAWKADSSPVKAGVETTTPSKQSNNKYAASSYLSLTPEQWKSHRSYSCQVTHEGSTVEKTVAPTECS

SEQ ID NO: 302 - protein, 231 aa, Homo sapiens
QVQLQQWGAGLLKPSETLSLTCAVYGGSFSAYYWNWIRQPPGKGLEWIGEINHSGRTDYNPSLKSRVTISVDTSKKQFSLKLNSVTAADTAVYYCARGQLVPFDYWGQGTLVTVSSASTKGPSVFPLAPSSKSTSGGTAALGCLVKDYFPEPVTVSWNSGALTSGVHTFPAVLQSSGLYSHSSVVTVPSSSLGTQTYICNVNHKPSNTKVDKKVEPKSCAADEVDHHHHHH

SEQ ID NO: 303 - protein, 680 aa, Homo sapiens
QEDEDGDYEELVLALRSEEDGLAEAPEHGTTATFHRCAKDPWRLPGTYVVVLKEETHLSQSERTARRLQAQAARRGYLTKILHVFHGLLPGFLVKMSGDLLELALKLPHVDYIEEDSSVFAQSIPWNLERITPPRYRADEYQPPDGGSLVEVYLLDTSIQSDHREIEGRVMVTDFENVPEEDGTRFHRQASKCDSHGTHLAGVVSGRDAGVAKGASMRSLRVLNCQGKGTVSGTLIGLEFIRKSQLVQPVGPLVVLLPLAGGYSRVLNAACQRLARAGVVLVTAAGNFRDDACLYSPASAPEVITVGATNAQDQPVTLGTLGTNFGRCVDLFAPGEDIIGASSDCSTCFVSQSGTSQAAAHVAGIAAMMLSAEPELTLAELRQRLIHFSAKDVINEAWFPEDQRVLTPNLVAALPPSTHGAGWQLFCRTVWSAHSGPTRMATAIARCAPDEELLSCSSFSRSGKRRGERMEAQGGKLVCRAHNAFGGEGVYAIARCCLLPQANCSVHTAPPAEASMGTRVHCHQQGHVLTGCSSHWEVEDLGTHKPPVLRPRGQPNQCVGHREASIHASCCHAPGLECKVKEHGIPAPQEQVTVACEEGWTLTGCSALPGTSHVLGAYAVDNTCVVRSRDVSTTGSTSEEAVTAVAICCRSRHLAQASQELQGSSDYKDDDKHHHHHHHH

SEQ ID NO: 304 - protein, 680 aa, Homo sapiens
RRRRRRRRRRRRLRRRRRRRRRRRRRRHRRRRRFRRCRRRPWRRPGRYVVVLRRRRRRSRSRETAEELQRRAREEGRRTKIRRRFRGLLPGFLVRMRRRLRRLARRLPRVRYIEEDSSVFRQRIPRNRREIRPPRYRARRRRPPRGGRRVEVYLLDTRIRRRHEEIRGRVRRRRFRRRPRRRRREREERRRRCDRRGTHLAGVVSGERAGVARRARMRSLEVLNCRGRGRVSGTLIGLERIERRRRRRPRRPLVVLLPLAGRYSEVLNRACRRLAERGVVLVTAAGNFEDDACRYSPARAPEVITVGATNRRRRPVRRGRRGTNFGRCVDLFAPGRRIIGASSRCSRCRRRRSGTSQAAAHVAGIAARMLRRRPRLRRARLRQELRRRSRRRRIRRRRFPRRRERLTPRLVARLPPRRRRRGRRLFCRTVWSRRSGPRERARAIAECAPREELLSCSSFSRSGKRRGERMERQGGKLVCRAHNARRGRGVYAIARCCLLPQARCSVHRAPPARRRRGTEVRCRRRGHVLTGCSSHWRRRDRGTRKPPRLRPEGRPRQCVGHREASIHASCCHAPGLECRRRRRRIPAPRERVTVRCRRGWTLTGCSALPGTSHVLGAYARDNTCVVRSEDRRRRRRRRRERVTAVAICCESEHLAQASQELQGSSDYKDDDKHHHHHHHH

SEQ ID NO: 305 - protein, 14 aa, Homo sapiens
TGTSSDVGGYNSVS

SEQ ID NO: 306 - protein, 7 aa, Homo sapiens
EVSNRPS

SEQ ID NO: 307 - protein, 9 aa, Homo sapiens
SSYTSTSMV

SEQ ID NO: 308 - protein, 5 aa, Homo sapiens
SYGIS

SEQ ID NO: 309 - protein, 17 aa, Homo sapiens
WISAYNGNTNYAQKVQG

SEQ ID NO: 310 - protein, 6 aa, Homo sapiens
GYGMDV

SEQ ID NO: 311 - protein, 14 aa, Homo sapiens
TGTSSDVGRYNSVS

SEQ ID NO: 312 - protein, 7 aa, Homo sapiens
EVSNRPS

SEQ ID NO: 313 - protein, 9 aa, Homo sapiens
SSYTSSSVV

SEQ ID NO: 314 - protein, 17 aa, Homo sapiens
WISAYNGNTNYAEKLQG

SEQ ID NO: 315 - protein, 6 aa, Homo sapiens
GYVMDV

SEQ ID NO: 316 - protein, 14 aa, Homo sapiens
TGTSSDVGAYNSVS

SEQ ID NO: 317 - protein, 9 aa, Homo sapiens
SSYTSTNMV

SEQ ID NO: 318 - protein, 17 aa, Homo sapiens
WVSAYNGNTNYAQKFQG

SEQ ID NO: 319 - protein, 9 aa, Homo sapiens
NSYTSTSMV

SEQ ID NO: 320 - protein, 17 aa, Homo sapiens
WVSFYNGNTNYAQKLQG

SEQ ID NO: 321 - protein, 7 aa, Homo sapiens
EVTNRPS

SEQ ID NO: 322 - protein, 14 aa, Homo sapiens
TGTNSDVGGYNSVS

SEQ ID NO: 323 - protein, 17 aa, Homo sapiens
WISVYNGNTNYAQKVQG

SEQ ID NO: 324 - protein, 17 aa, Homo sapiens
WISFYNGNTNYAQKVQG

SEQ ID NO: 325 - protein, 13 aa, Homo sapiens
SGSSSNIGNNFVS

SEQ ID NO: 326 - protein, 7 aa, Homo sapiens
DYNKRPS

SEQ ID NO: 327 - protein, 11 aa, Homo sapiens
GTWDSSLSGYV

SEQ ID NO: 328 - protein, 5 aa, Homo sapiens
SFGMH

SEQ ID NO: 329 - protein, 17 aa, Homo sapiens
LIWNDGSNKYYADSVKG

SEQ ID NO: 330 - protein, 13 aa, Homo sapiens
AIAALYYYYGMDV

SEQ ID NO: 331 - protein, 7 aa, Homo sapiens
DSNKRPS

SEQ ID NO: 332 - protein, 11 aa, Homo sapiens
GTWDSSLSAYV

SEQ ID NO: 333 - protein, 5 aa, Homo sapiens
SYGMH

SEQ ID NO: 334 - protein, 17 aa, Homo sapiens
LIWHDGSNTYYVDSVKG

SEQ ID NO: 335 - protein, 13 aa, Homo sapiens
GIAVAYYYYGMDV

SEQ ID NO: 336 - protein, 17 aa, Homo sapiens
LIWSDGSDEYYADSVKG

SEQ ID NO: 337 - protein, 11 aa, Homo sapiens
GTWDSSLSSYV

SEQ ID NO: 338 - protein, 17 aa, Homo sapiens
LIWSDGSDKYYADSVKG

SEQ ID NO: 339 - protein, 13 aa, Homo sapiens
SGSSSNIGSKTVN

SEQ ID NO: 340 - protein, 7 aa, Homo sapiens
SNNRRPS

SEQ ID NO: 341 - protein, 10 aa, Homo sapiens
AAWDDSLNWV

SEQ ID NO: 342 - protein, 4 aa, Homo sapiens
YWMS

SEQ ID NO: 343 - protein, 17 aa, Homo sapiens
NIKQDGSEKYYVDSVKG

SEQ ID NO: 344 - protein, 10 aa, Homo sapiens
ESNWGFAFDI

SEQ ID NO: 345 - protein, 13 aa, Homo sapiens
SGSSSNIGSNTVN

SEQ ID NO: 346 - protein, 5 aa, Homo sapiens
RYWMS

SEQ ID NO: 347 - protein, 17 aa, Homo sapiens
NIKHDGSEKYYVDSVKG

SEQ ID NO: 348 - protein, 10 aa, Homo sapiens
ESNWGFAFDV

SEQ ID NO: 349 - protein, 7 aa, Homo sapiens
RNNQRPL

SEQ ID NO: 350 - protein, 5 aa, Homo sapiens
SYWMS

SEQ ID NO: 351 - protein, 5 aa, Homo sapiens
NFWMS

SEQ ID NO: 352 - protein, 10 aa, Homo sapiens
RASQSISYLN

SEQ ID NO: 353 - protein, 6 aa, Homo sapiens
AASLQS

SEQ ID NO: 354 - protein, 8 aa, Homo sapiens
QQSYSPIT

SEQ ID NO: 355 - protein, 11 aa, Homo sapiens
RASQSISIYLN

SEQ ID NO: 356 - protein, 7 aa, Homo sapiens
AAASLQS

SEQ ID NO: 357 - protein, 9 aa, Homo sapiens
QQSYSAPIT

SEQ ID NO: 358 - protein, 11 aa, Homo sapiens
RASQSISSYLN

SEQ ID NO: 359 - protein, 7 aa, Homo sapiens
AASSLQS

SEQ ID NO: 360 - protein, 9 aa, Homo sapiens
QQSYSSPIT

SEQ ID NO: 361 - protein, 5 aa, Homo sapiens
SYAMN

SEQ ID NO: 362 - protein, 16 aa, Homo sapiens
TISGSGNTYYADSVKG

SEQ ID NO: 363 - protein, 12 aa, Homo sapiens
KFVLMVYAMLDY

SEQ ID NO: 364 - protein, 17 aa, Homo sapiens
TISGSGGNTYYADSVKG

SEQ ID NO: 365 - protein, 17 aa, Homo sapiens
TISGSGDNTYYADSVKG

SEQ ID NO: 366 - protein, 10 aa, Homo sapiens
GYSLTSYGIS

SEQ ID NO: 367 - protein, 10 aa, Homo sapiens
GYALTSYGIS

SEQ ID NO: 368 - protein, 10 aa, Homo sapiens
GYTLTSYGIS

SEQ ID NO: 369 - protein, 10 aa, Homo sapiens
GYSFTSYGIS

SEQ ID NO: 370 - protein, 10 aa, Homo sapiens
GYTFPSYGIS

SEQ ID NO: 371 - protein, 10 aa, Homo sapiens
GFTFSSYWMS

SEQ ID NO: 372 - protein, 10 aa, Homo sapiens
GFTFSRYWMS

SEQ ID NO: 373 - protein, 10 aa, Homo sapiens
GLTFSNFWMS

SEQ ID NO: 374 - protein, 10 aa, Homo sapiens
GFTFSSYAMN

SEQ ID NO: 375 - protein, 10 aa, Homo sapiens
GFTFNSFGMH

SEQ ID NO: 376 - protein, 10 aa, Homo sapiens
GFTFRSYGMH

SEQ ID NO: 377 - protein, 16 aa, Homo sapiens
NIKQDGSEKYVDSVKG

SEQ ID NO: 378 - protein, 16 aa, Homo sapiens
NIKHDGSEKYVDSVKG

SEQ ID NO: 379 - protein, 16 aa, Homo sapiens
TISGSGDNTYADSVKG

SEQ ID NO: 380 - protein, 16 aa, Homo sapiens
TISGSGGNTYADSVKG

SEQ ID NO: 381 - protein, 16 aa, Homo sapiens
LIWNDGSNKYADSVKG

SEQ ID NO: 382 - protein, 16 aa, Homo sapiens
LIWSDGSDEYADSVKG

SEQ ID NO: 383 - protein, 16 aa, Homo sapiens
LIWSDGSDKYADSVKG

SEQ ID NO: 384 - protein, 16 aa, Homo sapiens
LIWHDGSNTYVDSVKG

SEQ ID NO: 385 - protein, 10 aa, Homo sapiens
ESNWGFAFDI

SEQ ID NO: 386 - protein, 10 aa, Homo sapiens
ESNWGFAFDV

SEQ ID NO: 387 - protein, 6 aa, Homo sapiens
GYVMDV

SEQ ID NO: 388 - protein, 11 aa, Homo sapiens
RASQSISIYLN

SEQ ID NO: 389 - protein, 14 aa, Homo sapiens
TGTNSDVGGYNSVS

SEQ ID NO: 390 - protein, 14 aa, Homo sapiens
TGTSSDVGAYNSVS

SEQ ID NO: 391 - protein, 14 aa, Homo sapiens
TGTSSDVGRYNSVS

SEQ ID NO: 392 - protein, 7 aa, Homo sapiens
RNNQRPL

SEQ ID NO: 393 - protein, 7 aa, Homo sapiens
AAASLQS

SEQ ID NO: 394 - protein, 9 aa, Homo sapiens
QQSYSAPIT

SEQ ID NO: 395 - protein, 9 aa, Homo sapiens
NSYTSTSMV

SEQ ID NO: 396 - protein, 9 aa, Homo sapiens
SSYTSSSVV

SEQ ID NO: 397 - protein, 10 aa, Homo sapiens
AAWDDSLNWV

SEQ ID NO: 398 - protein, 11 aa, Homo sapiens
GTWDSSLSSYV

SEQ ID NO: 399 - protein, 11 aa, Homo sapiens
GTWDSSLSAYV

SEQ ID NO: 400 - protein, 116 aa, Homo sapiens
QVQLQESGPGLVKPSETLSLTCTVSGGSISSYYWSWIRQPPGKGLEWIGYIYYSGSTNYNPSLKSRVTISVDTSKNQFSLKLSSVTAADTAVYYCARYSSGWFDYWGQGTLVTVSS

SEQ ID NO: 401 - protein, 118 aa, Homo sapiens
EVQLVESGGGLVQPGGSLRLSCVVSGFTFSSYWMSWVRQAPGKGLEWVANIKQDGSEKYYVDSVKGRFTISRDNAKNSLYLQMNSLRAEDTAVYYCARESNWGFAFDIWGQGTMVTVS

SEQ ID NO: 402 - protein, 115 aa, Homo sapiens
EVQLVESGGGLVQPGGSLRLSCAASGFTFSSYWMSWVRQAPGKGLEWVANIKQDGSEKYYVDSVKGRFTISRDNAKNSLYLQMNSLRAEDTAVYYCARNWGAFDIWGQGTMVTVS

SEQ ID NO: 403 - protein, 6 aa, Homo sapiens
ENLYFQ

SEQ ID NO: 404-417 - skipped (14 entries)

SEQ ID NO: 418 - DNA, 363 bp, Homo sapiens
  source 1..363: mol_type = unassigned DNA
caggtgcaggtggtgcagtctggggctgaggtgaagaagcctggggcctcagtgaaggtctcctgcaaggcttctggatacaccttcaccggctactatatacactgggtgcgacaggcccctggacaagggcttgagtggatgggatggatcaaccctcacagtggtggcgcaaactatgcacagaagtttcagggcagggtcaccatgaccagggacacgtccatcagcacagcctacatggagctgagcaggctgagatctgacgacacggccgtgtattactgtgcgagaggcaactggaactacgactactacggtatggacgtctggggccaagggaccacggtcaccgtctcctca

SEQ ID NO: 419 - protein, 121 aa, Homo sapiens
QVQVVQSGAEVKKPGASVKVSCKASGYTFTGYYIHWVRQAPGQGLEWMGWINPHSGGANYAQKFQGRVTMTRDTSISTAYMELSRLRSDDTAVYYCARGNWNYDYYGMDVWGQGTTVTVSS

SEQ ID NO: 420 - DNA, 321 bp, Homo sapiens
  source 1..321: mol_type = unassigned DNA
gacatccagatgacccagtctccatcctccctgtctgcatctgtaggagacagagtcaccatcacttgccgggcgagtcaggacattagcaattatttagcctggtatcagcagaaaccagggaaagttcctaagctcctgatctatgctgcatccactttgcaatcaggggtcccatctcggttcagtggcagtggatctgggacagatttcactctcaccatcagcagcctacagcctgaagatgttgcaacttatttctgtcaaaggtatcagattgccccattcactttcggccctgggaccaaggtggatatcaaa

SEQ ID NO: 421 - protein, 107 aa, Homo sapiens
DIQMTQSPSSLSASVGDRVTITCRASQDISNYLAWYQQKPGKVPKLLIYAASTLQSGVPSRFSGSGSGTDFTLTISSLQPEDVATYFCQRYQIAPFTFGPGTKVDIK

SEQ ID NO: 422 - DNA, 366 bp, Homo sapiens
  source 1..366: mol_type = unassigned DNA
caggtgcagctggtggagtctgggggaggcgtggtccagcctgggaggtccctgagactctcctgtgcagcgtctggattcaccttcagtagctatggcatgcactgggtccgccaggctccaggcaaggggctggagtgggtggcagttatctggtatgatggaagtactaaatactatgcagactccgtgaagggccgatccaccatctccagagacaattccaagaacacgctgtatctgcaaatgaacagcctgagagccgaggacacggctgtgtattactgtgcgaggtcagtggctggttaccactactactacggtatggacgtctggggccaagggaccacggtcaccgtctcctca

SEQ ID NO: 423 - protein, 122 aa, Homo sapiens
QVQLVESGGGVVQPGRSLRLSCAASGFTFSSYGMHWVRQAPGKGLEWVAVIWYDGSTKYYADSVKGRSTISRDNSKNTLYLQMNSLRAEDTAVYYCARSVAGYHYYYGMDVWGQGTTVTVSS

SEQ ID NO: 424 - DNA, 324 bp, Homo sapiens
  source 1..324: mol_type = unassigned DNA
tcttctgagctgactcaggaccctgctgtgtctgtggccttgggacagacagtcaggatcacatgccaaggagacagcctcagaggctattatgcaacctggtaccagcagaagccaagacaggcccctgtacttgtcatctatggtaaaaactaccggccctcagggatcccagaccgattctctggctccacctcaggaaacacagcttccttgaccatcactggggctcaggcggaagatgaggctgactattactgtaactcccgggacagcattggtaaccatctggtgttcggcggagggaccaagctgaccgtccta

SEQ ID NO: 425 - protein, 108 aa, Homo sapiens
SSELTQDPAVSVALGQTVRITCQGDSLRGYYATWYQQKPRQAPVLVIYGKNYRPSGIPDRFSGSTSGNTASLTITGAQAEDEADYYCNSRDSIGNHLVFGGGTKLTVL

SEQ ID NO: 426 - DNA, 366 bp, Homo sapiens
  source 1..366: mol_type = unassigned DNA
caggtgcagctggtggagtctgggggaggcgtggtccagcctgggaggtccctgagactctcctgtgcagcgtctggattcaccttcagtagctatggcttgcactgggtccgccaggctccaggcaaggggctggagtgggtggcagttatatggttagatggaagtaataaatactatgcagactccgtgaagggccgatccaccatctccagagacaattccaagaacacgctgtatctgcaaatgaacagcctgagagccgaggacacggctgtgtattactgtgcgaggtcagtggctggttaccactactactacggtatggacgtctggggccaagggaccacggtcaccgtctcctca

SEQ ID NO: 427 - protein, 122 aa, Homo sapiens
QVQLVESGGGVVQPGRSLRLSCAASGFTFSSYGLHWVRQAPGKGLEWVAVIWLDGSNKYYADSVKGRSTISRDNSKNTLYLQMNSLRAEDTAVYYCARSVAGYHYYYGMDVWGQGTTVTVSS

SEQ ID NO: 428 - DNA, 324 bp, Homo sapiens
  source 1..324: mol_type = unassigned DNA
tcttctgagctgactcaggaccctgctgtgtctgtggccttgggacagacagtcaggatcacatgccaaggagacagcctcagaagttattatggaagctggtaccagcagaagccaagacaggcccctgtacttgtcatctttggtaaaaacaaccggccctcagggatcccagaccgattctctggctccacctcaggaaacacagcttccttgaccatcactggggctcaggcggaagatgaggctgactattactgtaactcacgggacatcattggtgaccatctgctgttcggcggagggaccaagctgaccgtccta

SEQ ID NO: 429 - protein, 108 aa, Homo sapiens
SSELTQDPAVSVALGQTVRITCQGDSLRSYYGSWYQQKPRQAPVLVIFGKNNRPSGIPDRFSGSTSGNTASLTITGAQAEDEADYYCNSRDIIGDHLLFGGGTKLTVL

SEQ ID NO: 430 - DNA, 366 bp, Homo sapiens
  source 1..366: mol_type = unassigned DNA
caggtgcagctggtggagtctgggggaggcgtggtccagtctgggaggtccctgagactctcctgtgcagcgtctggattcaccttcaggaactatggcatgcactgggtccgccaggctccaggcaaggggctggagtgggtggcagttatatggtttgatggaagtaataaatactatgcagactccgtgaagggccgatccaccatctccagagacaattccaagaacacgctgtatctgctaatgaacagcctgagagccgaggacacggctgtgtattactgtgcgaggtcagtggctggttaccactactactacggtatggacgtctggggccaagggaccacggtcaccgtctcctca

SEQ ID NO: 431 - protein, 122 aa, Homo sapiens
QVQLVESGGGVVQSGRSLRLSCAASGFTFRNYGMHWVRQAPGKGLEWVAVIWFDGSNKYYADSVKGRSTISRDNSKNTLYLLMNSLRAEDTAVYYCARSVAGYHYYYGMDVWGQGTTVTVSS

SEQ ID NO: 432 - DNA, 324 bp, Homo sapiens
  source 1..324: mol_type = unassigned DNA
tcttctgagctgactcaggaccctgctgtgtctgtggccttgggacagacagtcaggatcacatgccagggagacagcctcagaagctattatgcaagctggtaccagcagaagccaagacaggcccctgtacttgtcatctatggtaaaaacaaccggccctcagggatcccagaccgaatctctggctccacctcaggaaacacagcttccttgaccatcactggggctcaggcggaagatgaggctgactattactgtaaatcccgggacatcattggtgaccatctggtgttcggcggagggaccaaactgaccgtccta

SEQ ID NO: 433 - protein, 108 aa, Homo sapiens
SSELTQDPAVSVALGQTVRITCQGDSLRSYYASWYQQKPRQAPVLVIYGKNNRPSGIPDRISGSTSGNTASLTITGAQAEDEADYYCKSRDIIGDHLVFGGGTKLTVL

SEQ ID NO: 434 - DNA, 342 bp, Homo sapiens
  source 1..342: mol_type = unassigned DNA
caggtgcagctggtggagtctgggggaggcgtggtccagcctgggaggtccctgagactctcctgtgcagcgtctggattcaccttcagtagctatggcatgcactgggtccgccaggctccaggcaaggggctggagtgggtggcagttatatggtatgatggaagtaataaatactatgcagactccgtgaagggccgattcaccatctccagagacaattccaagaacacgctgtatctgcaaatgaacagcctgagagccgaggacacggctgtgtattactgtgtgagagatcggggactggactggggccagggaaccctggtcaccgtctcctca

SEQ ID NO: 435 - protein, 114 aa, Homo sapiens
QVQLVESGGGVVQPGRSLRLSCAASGFTFSSYGMHWVRQAPGKGLEWVAVIWYDGSNKYYADSVKGRFTISRDNSKNTLYLQMNSLRAEDTAVYYCVRDRGLDWGQGTLVTVSS

SEQ ID NO: 436 - DNA, 324 bp, Homo sapiens
  source 1..324: mol_type = unassigned DNA
tcttctgagctgactcaggaccctgctgtgtctgtggccttgggacagacagtcaggatcacatgccaaggagacagcctcagaggctattatgcaagctggtaccagcagaagccaagacaggcccctgtacttgtcatctatggtaaaaacaaccggccctcagggatcccagaccgattctctggctccacctcaggaaacacagcttccttgaccatcactggggctcaggcggaagatgaggctgactattactgtaagtcccgggacagcagtggtgaccatctggtgttcggcggagggaccaagctgaccgtccta

SEQ ID NO: 437 - protein, 108 aa, Homo sapiens
SSELTQDPAVSVALGQTVRITCQGDSLRGYYASWYQQKPRQAPVLVIYGKNNRPSGIPDRFSGSTSGNTASLTITGAQAEDEADYYCKSRDSSGDHLVFGGGTKLTVL

SEQ ID NO: 438 - DNA, 366 bp, Homo sapiens
  source 1..366: mol_type = unassigned DNA
caggtgcaggtggtggagtctgggggaggcgtggtccagcctggggggtccctgagactctcctgtgcagcgtctggattcaccttcagtaactatggcatgcactgggtccgccaggctccaggcaaggggctggagtgggtggcagttatttggtatgatggaagtagtaaatactatgcagactccgtgaagggccgatccaccatctccagagacaattccaagaacacggtgtatctgcaaatgaacagcctgagagccgaggacacggctgtgtattactgtgcgaggtcagtggctggttaccactactactacggtatggacgtctggggccaagggaccacggtcaccgtctcctca

SEQ ID NO: 439 - protein, 122 aa, Homo sapiens
QVQVVESGGGVVQPGGSLRLSCAASGFTFSNYGMHWVRQAPGKGLEWVAVIWYDGSSKYYADSVKGRSTISRDNSKNTVYLQMNSLRAEDTAVYYCARSVAGYHYYYGMDVWGQGTTVTVSS

SEQ ID NO: 440 - DNA, 324 bp, Homo sapiens; identical to SEQ ID NO: 436
  source 1..324: mol_type = unassigned DNA

SEQ ID NO: 441 - protein, 108 aa, Homo sapiens; identical to SEQ ID NO: 437

SEQ ID NO: 442 - DNA, 366 bp, Homo sapiens
  source 1..366: mol_type = unassigned DNA
caggtgcagctggtggagtctgggggaggcgtggtccagcctgggaggtccctgagtctctcctgtgcagcgtctggattcaccttcagtagctatggcatgcactgggtccgccaggctccaggcaaggggctggagtgggtggcagttatatggtatgatggaagttataaagactatgcagactccgtgaagggccgatccaccatctccagagacaactccaagaacacgctgtatctgcaaatgaacagcctgagagccgaggacacggctgtgtattattgtgcgaggtcagtggctggttaccactactactacggtatggacgtctggggccaagggaccacggtcaccgtctcctca

SEQ ID NO: 443 - protein, 122 aa, Homo sapiens
QVQLVESGGGVVQPGRSLSLSCAASGFTFSSYGMHWVRQAPGKGLEWVAVIWYDGSYKDYADSVKGRSTISRDNSKNTLYLQMNSLRAEDTAVYYCARSVAGYHYYYGMDVWGQGTTVTVSS

SEQ ID NO: 444 - DNA, 324 bp, Homo sapiens
  source 1..324: mol_type = unassigned DNA
tcttctgagctgactcaggaccctgctgtgtctgtggccttgggacagacagtcaggatcacatgccaaggagacagcctcagaacctattatgcaagctggtaccagcagaagccaagacaggcccctattcttgtcatctatggtaaaaacaaccggccctcagggatcccagaccgattctctggctccacctcaggaatcacagcttccttgaccatcactggggctcaggcggaagatgaggctgactattactgtaaatcccgggacatcattggtaaccatctgctgttcggcggagggactaagctgaccgtccta

SEQ ID NO: 445 - protein, 108 aa, Homo sapiens
SSELTQDPAVSVALGQTVRITCQGDSLRTYYASWYQQKPRQAPILVIYGKNNRPSGIPDRFSGSTSGITASLTITGAQAEDEADYYCKSRDIIGNHLLFGGGTKLTVL

SEQ ID NO: 446 - DNA, 375 bp, Homo sapiens
  source 1..375: mol_type = unassigned DNA
caggtgcagctggtggcgtctgggggaggcgtggtccagcctgggaggtccctgagactctcctgtgcagcgtctggattcaccctcagtagctatggcatgcactgggtccgccaggctccaggccaggggctggagtgggtggcagtcatatggtatgatggaagtaacaaatactatgcagcctccgtgaagggccgattcaccatctccagagacaattccaagaacacgctgtatctgcaaatgaacagtctgagagccgaggacacggctgtgtattactgtgcgagagggggtggttcggggagtcatcgctactactactacggtatggacgtctggggccaagggaccacggtcaccgtctcctca

SEQ ID NO: 447 - protein, 125 aa, Homo sapiens
QVQLVASGGGVVQPGRSLRLSCAASGFTLSSYGMHWVRQAPGQGLEWVAVIWYDGSNKYYAASVKGRFTISRDNSKNTLYLQMNSLRAEDTAVYYCARGGGSGSHRYYYYGMDVWGQGTTVTVSS

SEQ ID NO: 448 - DNA, 324 bp, Homo sapiens; identical to SEQ ID NO: 444
  source 1..324: mol_type = unassigned DNA

SEQ ID NO: 449 - protein, 108 aa, Homo sapiens; identical to SEQ ID NO: 445

SEQ ID NO: 450 - DNA, 366 bp, Homo sapiens
  source 1..366: mol_type = unassigned DNA
caggtgcaagtggtggagtctgggggaggcgtggtccagcctgggaggtccctgagactctcctgtgcagcgtctggattcaccttcagtaactatggcatgcactgggtccgccaggctccaggcaaggggctggagtgggtggcagttatatggtatgatggaggtaataaatactatgcagactccgtgaagggccgatccatcatctccagagacaattccaagagcacgctgtatctgcaaatgaacagcctgagagccgaggacacggctgtttattattgtgcgaggtcagtggctggttaccattattactacggtatggacgtctggggccaagggaccacggtcaccgtcgcctca

SEQ ID NO: 451 - protein, 122 aa, Homo sapiens
QVQVVESGGGVVQPGRSLRLSCAASGFTFSNYGMHWVRQAPGKGLEWVAVIWYDGGNKYYADSVKGRSIISRDNSKSTLYLQMNSLRAEDTAVYYCARSVAGYHYYYGMDVWGQGTTVTVAS

SEQ ID NO: 452 - DNA, 327 bp, Homo sapiens
  source 1..327: mol_type = unassigned DNA
cagtctgccctgactcagcctgcctccgtgtctgggtctcctggacagtcgatcaccatctcctgcactggaaccagcagtgacgttggtggttataactctgtctcctggtaccaacagcacccaggcaaaccccccaaactcatgatttatgaggtcagtaatcggccctcagggatttctaatcgcttctctggctccaagtctggcaacacggcctccctgaccatctctgggctccaggctgaggacgaggctgattatttctgcagctcatatacaagcaccagcatggtcttcggcggagggaccaagctggccgtccta

SEQ ID NO: 453 - protein, 109 aa, Homo sapiens
QSALTQPASVSGSPGQSITISCTGTSSDVGGYNSVSWYQQHPGKPPKLMIYEVSNRPSGISNRFSGSKSGNTASLTISGLQAEDEADYFCSSYTSTSMVFGGGTKLAVL

SEQ ID NO: 454 - DNA, 366 bp, Homo sapiens; identical to SEQ ID NO: 450
  source 1..366: mol_type = unassigned DNA

SEQ ID NO: 455 - protein, 122 aa, Homo sapiens; identical to SEQ ID NO: 451

SEQ ID NO: 456 - DNA, 324 bp, Homo sapiens
  source 1..324: mol_type = unassigned DNA
tcttctgagctgactcaggaccctgctgtgtctgtggccttgggacagacagtcaggatcacatgccaaggagacagcctcagaggctattatgcaagctggtaccagcagaagccaagacaggcccctgtacttgtcatctatggtaaaaacaaccggccctcagggatcccagaccgattctctggctccacgtcaggaaacacagcttccttgaccatcactggggctcaggcggaagatgaggctgactattactgtaactcccgggacaacattggtgaccatctggtgttcggcggagggaccaagctgaccgtccta

SEQ ID NO: 457 - protein, 108 aa, Homo sapiens
SSELTQDPAVSVALGQTVRITCQGDSLRGYYASWYQQKPRQAPVLVIYGKNNRPSGIPDRFSGSTSGNTASLTITGAQAEDEADYYCNSRDNIGDHLVFGGGTKLTVL

SEQ ID NO: 458 - DNA, 381 bp, Homo sapiens
  source 1..381: mol_type = unassigned DNA
gaggtgcagctggtggagtctgggggaggcttggtccagcctggggggtccctgagactctcctgtgcagcctccggattcacctttagtagctattggatgagctgggtccgccaggctccagggaaggggctggagtgggtggccagcataaaacaagatggaagtgagaaatactatgtggactctgtgaagggccgattcaccatctccagagacaacgccaggaactcactgtatctgcaaatgaacagcctgagagccgaggacacggctgtgtattactgtgcgagagatcttgtattaatggtgtatgatatagactactactactacggtatggacgtctggggccaagggaccacggtcaccgtctcctca

SEQ ID NO: 459 - protein, 127 aa, Homo sapiens
EVQLVESGGGLVQPGGSLRLSCAASGFTFSSYWMSWVRQAPGKGLEWVASIKQDGSEKYYVDSVKGRFTISRDNARNSLYLQMNSLRAEDTAVYYCARDLVLMVYDIDYYYYGMDVWGQGTTVTVSS

SEQ ID NO: 460 - DNA, 336 bp, Homo sapiens
  source 1..336: mol_type = unassigned DNA
gatattgtgatgactcagtctccactctccctgcccgtcacccctggagagccggcctccatctcctgcaggtctagtcagagcctcctgcatagtaatggatacaactatttggattggtacctgcagaagccagggcagtctccacagctcctgatctatttgggttctaatcgggcctccggggtccctgacaggttcagtggcagtggatcaggcacagattttacactgaaaatcagcagagtggaggctgaggatgttggggtttattactgcatgcaagctctacaaactccgctcactttcggcggagggaccaaggtagagatcaaa

SEQ ID NO: 461 - protein, 112 aa, Homo sapiens
DIVMTQSPLSLPVTPGEPASISCRSSQSLLHSNGYNYLDWYLQKPGQSPQLLIYLGSNRASGVPDRFSGSGSGTDFTLKISRVEAEDVGVYYCMQALQTPLTFGGGTKVEIK

SEQ ID NO: 462 - DNA, 381 bp, Homo sapiens
  source 1..381: mol_type = unassigned DNA
gaggtgcagctggtggagtctgggggaggcttggtccagcctggggggtccctgagactctcctgtgcagcctccggattcacctttagtaactattggatgagctgggtccgccaggctccagggaaggggctggagtgggtggccagcataaaacaagatggaagtgagaaatactatgtggactctgtgaagggccgattcgccatctccagagacaacgccaagaactcactgtttctgcaaatgaacagcctgagagccgaggacacggctgtgtattactgtgcgagagatcttgtactaatggtgtatgatatagactactactactacggtatggacgtctggggccaagggaccacggtcaccgtctcctca

SEQ ID NO: 463 - protein, 127 aa, Homo sapiens
EVQLVESGGGLVQPGGSLRLSCAASGFTFSNYWMSWVRQAPGKGLEWVASIKQDGSEKYYVDSVKGRFAISRDNAKNSLFLQMNSLRAEDTAVYYCARDLVLMVYDIDYYYYGMDVWGQGTTVTVSS

SEQ ID NO: 464 - DNA, 336 bp, Homo sapiens
  source 1..336: mol_type = unassigned DNA
gatattgtgatgactcagtctccactctccctgcctgtcacccctggagagccggcctccatctcttgcaggtctagtcagagcctcctgcatagtaatgggtacaactatttggattggtacctgcagaagccagggcagtctccacagctcctgatctatttgggttctaatcgggcctccggggtccctgacaggttcagtggcagtggatcaggcacacatcttacactgaaaatcagcagagtggaggctgaggatgttggagtttattactgcatgcaaactctacaaactccgctcactttcggcggagggaccaaggtggagatcaaa

SEQ ID NO: 465 - protein, 112 aa, Homo sapiens
DIVMTQSPLSLPVTPGEPASISCRSSQSLLHSNGYNYLDWYLQKPGQSPQLLIYLGSNRASGVPDRFSGSGSGTHLTLKISRVEAEDVGVYYCMQTLQTPLTFGGGTKVEIK

SEQ ID NO: 466 - DNA, 342 bp, Homo sapiens
  source 1..342: mol_type = unassigned DNA
caggtgcagctggtggagtctgggggaggcgtggcccagcctgggaggtccctgagactctcctgtgcagcgtctggattcaccttcagtagctatggcatgcactgggtccgccaggctccaggcaaggggctggagtgggtggcagttatatactatgatggaattaataaacactatgcagactccgtgaagggccgattcaccatctccagagacaattccaagaacacgctgtatctgcaaatgaacagcctgagagccgaggacacggctgtgtattactgtgcgagagatcggggactggactggggccagggaaccctggtcaccgtctcctca

SEQ ID NO: 467 - protein, 114 aa, Homo sapiens
QVQLVESGGGVAQPGRSLRLSCAASGFTFSSYGMHWVRQAPGKGLEWVAVIYYDGINKHYADSVKGRFTISRDNSKNTLYLQMNSLRAEDTAVYYCARDRGLDWGQGTLVTVSS

SEQ ID NO: 468 - DNA, 339 bp, Homo sapiens
  source 1..339: mol_type = unassigned DNA
gacatcgtgatgacccagtctccagactccctggctgtgtctctgggcgagagggccaccatcaactgcaagtccagccagagtgttttatacagctccaacagtaagaactacttagtttggtaccagcagaaaccaggacagcctcctaagctgctcatttactgggcctctacccgggaatccggggtccctgaccgattcagtggcagcgggtctgggacagatttcactctcaccatcagcagcctgcaggctgaagatgtggcagtttattactgtcaacaatattatagtactccgtggacgttcggccaagggaccaaggtggaaatcaaa

SEQ ID NO: 469 - protein, 113 aa, Homo sapiens
DIVMTQSPDSLAVSLGERATINCKSSQSVLYSSNSKNYLVWYQQKPGQPPKLLIYWASTRESGVPDRFSGSGSGTDFTLTISSLQAEDVAVYYCQQYYSTPWTFGQGTKVEIK

SEQ ID NO: 470 - DNA, 357 bp, Homo sapiens
  source 1..357: mol_type = unassigned DNA
gaggtgcagctggtggagtctgggggaggcttggtccagcctggggggtccctgagactctcctgtgcagcctctggactcacctttagtaacttttggatgagctgggtccgccaggctccagggaaggggctggagtgggtggccaacataaagcaagatggaaatgataaatactatgtggactctgtgaagggccgattcaccatctccagagacaacgccaagaattcactgtatctgcaaatgaacagcctgagagccgaggacacggctgtgtattactgtgcgagagagtcaaactggggatttgcttttgatatctggggccaagggacaatggtcaccgtctcttca

SEQ ID NO: 471 - protein, 119 aa, Homo sapiens
EVQLVESGGGLVQPGGSLRLSCAASGLTFSNFWMSWVRQAPGKGLEWVANIKQDGNDKYYVDSVKGRFTISRDNAKNSLYLQMNSLRAEDTAVYYCARESNWGFAFDIWGQGTMVTVSS

SEQ ID NO: 472 - DNA, 327 bp, Homo sapiens; identical to SEQ ID NO: 145
  source 1..327: mol_type = unassigned DNA

SEQ ID NO: 473 - protein, 109 aa, Homo sapiens; identical to SEQ ID NO: 33

SEQ ID NO: 474 - DNA, 357 bp, Homo sapiens
  source 1..357: mol_type = unassigned DNA
gaggtgcagctggtggagtctgggggaggtttggtccagcctggggggtccctgagactctcctgtgcagcctctggactcacctttagtaacttttggatgagctgggtccgccaggctccagggaaggggctggagtgggtggccaacataaagcaagatggaagtgagaaatactatgtggactctgtgaagggccgattcaccatctccagagacaacgccaagaattcactgtatctgcaaatgaacagcctgagagccgaggacacggctgtgtattactgtgcgagagagtcaaactggggatttgcttttgatatctggggccaagggacaatggtcaccgtctcttca

SEQ ID NO: 475 - protein, 119 aa, Homo sapiens
EVQLVESGGGLVQPGGSLRLSCAASGLTFSNFWMSWVRQAPGKGLEWVANIKQDGSEKYYVDSVKGRFTISRDNAKNSLYLQMNSLRAEDTAVYYCARESNWGFAFDIWGQGTMVTVSS

SEQ ID NO: 476 - DNA, 327 bp, Homo sapiens
  source 1..327: mol_type = unassigned DNA
cagtctgtgctgactcagccaccctcagcgtctgggacccccgggcagagggtcaccatctcttgttctggaagcagctccaacatcggaagtaaaactgtaaactggtaccagcagttcccaggaacggcccccaaactcctcatctatagtaataatcggcggccctcaggggtccctgaccgattctctggctccaagtctggcacctcagcctccctggccatcagtgggctccagtctgaggatgaggctgattattactgtgcaacatgggatgacagactgaattgggtgttcggcgcagggaccaagctgaccgtccta

SEQ ID NO: 477 - protein, 109 aa, Homo sapiens
QSVLTQPPSASGTPGQRVTISCSGSSSNIGSKTVNWYQQFPGTAPKLLIYSNNRRPSGVPDRFSGSKSGTSASLAISGLQSEDEADYYCATWDDRLNWVFGAGTKLTVL

SEQ ID NO: 478 - DNA, 366 bp, Homo sapiens
  source 1..366: mol_type = unassigned DNA
caggtcaccttgaaggagtctggtcctgtgctggtgaaacccacagagaccctcacgctgacctgcaccgtctctgggttctcactcagcaatgttagaatgggtgtgagctggatccgtcagcccccagggaaggccctggagtggcttgcacacattttttcgaatgacgaaaattcctacagaacatctctgaagagcaggctcaccatctccaaggacacctccaaaagccaggtggtccttaccatgaccaacatggaccctgtggacacagccacatattactgtgcacggatagtgggagctacaacggatgatgcttttgatatctggggccaagggacaatggtcaccgtctcttca

SEQ ID NO: 479 - protein, 122 aa, Homo sapiens
QVTLKESGPVLVKPTETLTLTCTVSGFSLSNVRMGVSWIRQPPGKALEWLAHIFSNDENSYRTSLKSRLTISKDTSKSQVVLTMTNMDPVDTATYYCARIVGATTDDAFDIWGQGTMVTVSS

SEQ ID NO: 480 - DNA, 324 bp, Homo sapiens
  source 1..324: mol_type = unassigned DNA
tcctatgtgctgactcagccaccctcggtgtcagtggccccaggacagacggccaggattacctgtgggggaaacaacattggaagtaaaagtgtgcactggtaccagcagaagccaggccaggcccctgtgctggtcgtctatgatgatagcgaccggccctcagggatccctgagcgattctctggctccaactctgggaacacggccaccctgaccatcagcagggtcgaagccggggatgaggccgacttttactgtcaggtgtgggatagtagtagtgatcctgtggtattcggcggagggaccaagctgaccgtccta

SEQ ID NO: 481 - protein, 108 aa, Homo sapiens
SYVLTQPPSVSVAPGQTARITCGGNNIGSKSVHWYQQKPGQAPVLVVYDDSDRPSGIPERFSGSNSGNTATLTISRVEAGDEADFYCQVWDSSSDPVVFGGGTKLTVL

SEQ ID NO: 482 - DNA, 381 bp, Homo sapiens
  source 1..381: mol_type = unassigned DNA
gaggtgcagctggtggagtctgggggaggcttggtccagcctggggggtccctgagactctcctgtgcagcctctggattcacctttagtaactattggatgacctgggtccgccaggctccagggaaggggctggagtgggtggccagcataaagcaagatggaagtgagagatactatgtggactctgtgaagggccgattcaccatctcccgagacaccgccaagaactctctgtatctccaaatgaacagcctgcgagccgaggacacggctgtgtattactgtgcgagacctcttgtactaatggtgtatgctctacactactactactacggtatggacgtctggggccacgggaccacggtcaccgtctcctca

SEQ ID NO: 483 - protein, 127 aa, Homo sapiens
EVQLVESGGGLVQPGGSLRLSCAASGFTFSNYWMTWVRQAPGKGLEWVASIKQDGSERYYVDSVKGRFTISRDTAKNSLYLQMNSLRAEDTAVYYCARPLVLMVYALHYYYYGMDVWGHGTTVTVSS

SEQ ID NO: 484 - DNA, 336 bp, Homo sapiens
  source 1..336: mol_type = unassigned DNA
gatattgtgatgactcagtctccactctccctgcccgtcacccctggagagccggcctccatctcctgcaggtctagtcagagcctcctgcatagtaatggatacaactatttggattggtacctgcagaagccagggcagtctccacagctcctgatctatttgggttctaatcgggcctccggggtccctgacaggttcagtggcagtggatcaggcacagattttacactgaaaatcagcagagtggaggctgaggatgttggggtttattactgcatgcaagctctacaaactccgctcactttcggcggagggaccaaggtggagatcaaa

SEQ ID NO: 485 - protein, 112 aa, Homo sapiens; identical to SEQ ID NO: 461

SEQ ID NO: 486 - protein, 100 aa, Homo sapiens
QVTLKESGPVLVKPTETLTLTCTVSGFSLSNARMGVSWIRQPPGKALEWLAHIFSNDEKSYSTSLKSRLTISKDTSKSQVVLTMTNMDPVDTATYYCARI

SEQ ID NO: 487 - protein, 98 aa, Homo sapiens
EVQLVESGGGLVQPGGSLRLSCAASGFTFSSYWMSWVRQAPGKGLEWVANIKQDGSEKYYVDSVKGRFTISRDNAKNSLYLQMNSLRAEDTAVYYCAR

SEQ ID NO: 488 - protein, 98 aa, Homo sapiens
QVQLVESGGGVVQPGRSLRLSCAASGFTFSSYGMHWVRQAPGKGLEWVAVIWYDGSNKYYADSVKGRFTISRDNSKNTLYLQMNSLRAEDTAVYYCAR

SEQ ID NO: 489 - protein, 93 aa, Homo sapiens
DIVMTQSPLSLPVTPGEPASISCRSSQSLLHSNGYNYLDWYLQKPGQSPQLLIYLGSNRASGVPDRFSGSGSGTDFTLKISRVEAEDVGVYYC

SEQ ID NO: 490 - protein, 94 aa, Homo sapiens
DIVMTQSPDSLAVSLGERATINCKSSQSVLYSSNNKNYLAWYQQKPGQPPKLLIYWASTRESGVPDRFSGSGSGTDFTLTISSLQAEDVAVYYC

SEQ ID NO: 491 - protein, 89 aa, Homo sapiens
QSVLTQPPSASGTPGQRVTISCSGSSSNIGSNTVNWYQQLPGTAPKLLIYSNNQRPSGVPDRFSGSKSGTSASLAISGLQSEDEADYYC

SEQ ID NO: 492 - protein, 87 aa, Homo sapiens
SYVLTQPPSVSVAPGKTARITCGGNNIGSKSVHWYQQKPGQAPVLVIYYDSDRPSGIPERFSGSNSGNTATLTISRVEAGDEADYYC

SEQ ID NO: 493 - protein, 49 aa, Homo sapiens
QVQLVQSGAEVKKPGASVKVSCKASGYTFTGYYMHWVRQAPGQGLEWMG

SEQ ID NO: 494 - protein, 98 aa, Homo sapiens; identical to SEQ ID NO: 488

SEQ ID NO: 495 - protein, 98 aa, Homo sapiens; identical to SEQ ID NO: 488

SEQ ID NO: 496 - protein, 88 aa, Homo sapiens
DIQMTQSPSSLSASVGDRVTITCRASQGISNYLAWYQQKPGKVPKLLIYAASTLQSGVPSRFSGSGSGTDFTLTISSLQPEDVATYYC

SEQ ID NO: 497 - protein, 90 aa, Homo sapiens
QSALTQPASVSGSPGQSITISCTGTSSDVGGYNYVSWYQQHPGKAPKLMIYEVSNRPSGVSNRFSGSKSGNTASLTISGLQAEDEADYYC

SEQ ID NO: 498 - protein, 87 aa, Homo sapiens
SSELTQDPAVSVALGQTVRITCQGDSLRSYYASWYQQKPGQAPVLVIYGKNNRPSGIPDRFSGSSSGNTASLTITGAQAEDEADYYC

SEQ ID NO: 499 - protein, 13 aa, Homo sapiens
SGSSSNIGSKTVN

SEQ ID NO: 500 - protein, 10 aa, Homo sapiens
GFTFSNYWMS

SEQ ID NO: 501 - protein, 17 aa, Homo sapiens
SIKQDGSEKYYVDSVKG

SEQ ID NO: 502 - protein, 18 aa, Homo sapiens
DLVLMVYDIDYYYYGMDV

SEQ ID NO: 503 - protein, 15 aa, Homo sapiens
RSSQSLLHSNGYNLD

SEQ ID NO: 504 - protein, 7 aa, Homo sapiens
LGSNRAS

SEQ ID NO: 505 - protein, 9 aa, Homo sapiens
MQTLQTPLT

SEQ ID NO: 506 - protein, 25 aa, Homo sapiens
QVTLKESGPVLVKPTETLTLTCTVS

SEQ ID NO: 507 - protein, 12 aa, Homo sapiens
GFSLSNARMGVS

SEQ ID NO: 508 - protein, 12 aa, Homo sapiens
GFSLSNVRMGVS

SEQ ID NO: 509 - protein, 14 aa, Homo sapiens
WIRQPPGKALEWLA

SEQ ID NO: 510 - protein, 25 aa, Homo sapiens [sequence omitted]

SEQ ID NO: 511 - protein, 10 aa, Homo sapiens
GFTFSSYWMS

SEQ ID NO: 512 - protein, 10 aa, Homo sapiens
GLTFSNFWMS

SEQ ID NO: 513 - protein, 10 aa, Homo sapiens
GFTFSNYWMT

SEQ ID NO: 514 - protein, 14 aa, Homo sapiens
WVRQAPGKGLEWVA

SEQ ID NO: 515 - protein, 25 aa, Homo sapiens
QVQLVESGGGVVQPGRSLRLSCAAS

SEQ ID NO: 516 - protein, 25 aa, Homo sapiens
QVQLVESGGGVAQPGRSLRLSCAAS

SEQ ID NO: 517 - protein, 10 aa, Homo sapiens
GFTFSSYGMH

SEQ ID NO: 518 - protein, 14 aa, Homo sapiens
WVRQAPGKGLEWVA

SEQ ID NO: 519 - protein, 16 aa, Homo sapiens
HIFSNDEKSYSTSLKS

SEQ ID NO: 520 - protein, 16 aa, Homo sapiens
HIFSNDENSYRTSLKS

SEQ ID NO: 521 - protein, 33 aa, Homo sapiens
RLTISKDTSKSQVVLTMTNMDPVDTATYYCARI

SEQ ID NO: 522 - protein, 11 aa, Homo sapiens
VGATTDDAFDI

SEQ ID NO: 523 - protein, 11 aa, Homo sapiens
WGQGTMVTVSS

SEQ ID NO: 524 - protein, 11 aa, Homo sapiens
WGQGTTVTVSS

SEQ ID NO: 525 - protein, 11 aa, Homo sapiens
WGHGTTVTVSS

SEQ ID NO: 526 - protein, 17 aa, Homo sapiens
NIKQDGSEKYYVDSVKG

SEQ ID NO: 527 - protein, 17 aa, Homo sapiens
NIKQDGNDKYYVDSVKG

SEQ ID NO: 528 - protein, 17 aa, Homo sapiens
SIKQDGSERYYVDSVKG

SEQ ID NO: 529 - protein, 32 aa, Homo sapiens
RFTISRDNAKNSLYLQMNSLRAEDTAVYYCAR

SEQ ID NO: 530 - protein, 32 aa, Homo sapiens
RFTISRDNARNSLYLQMNSLRAEDTAVYYCAR

SEQ ID NO: 531 - protein, 32 aa, Homo sapiens
RFAISRDNAKNSLFLQMNSLRAEDTAVYYCAR

SEQ ID NO: 532 - protein, 32 aa, Homo sapiens
RFTISRDTAKNSLYLQMNSLRAEDTAVYYCAR

SEQ ID NO: 533 - protein, 10 aa, Homo sapiens
ESNWGFAFDI

SEQ ID NO: 534 - protein, 18 aa, Homo sapiens
PLVLMVYALHYYYYGMDV

SEQ ID NO: 535 - protein, 17 aa, Homo sapiens
VIWYDGSNKYYADSVKG

SEQ ID NO: 536 - protein, 17 aa, Homo sapiens
VIYYDGINKHYADSVKG

SEQ ID NO: 537 - protein, 32 aa, Homo sapiens
RFTISRDNSKNTLYLQMNSLRAEDTAVYYCAR

SEQ ID NO: 538 - protein, 5 aa, Homo sapiens
DRGLD

SEQ ID NO: 539 - protein, 11 aa, Homo sapiens
WGQGTLVTVSS

SEQ ID NO: 540 - protein, 23 aa, Homo sapiens
DIVMTQSPLSLPVTPGEPASISC

SEQ ID NO: 541 - protein, 15 aa, Homo sapiens
WYLQKPGQSPQLLIY

SEQ ID NO: 542 - protein, 23 aa, Homo sapiens
DIVMTQSPDSLAVSLGERATINC

SEQ ID NO: 543 - protein, 17 aa, Homo sapiens
KSSQSVLYSSNNKNYLA

SEQ ID NO: 544 - protein, 17 aa, Homo sapiens
KSSQSVLYSSNSKNYLV

SEQ ID NO: 545 - protein, 15 aa, Homo sapiens
WYQQKPGQPPKLLIY

SEQ ID NO: 546 - protein, 22 aa, Homo sapiens
QSVLTQPPSASGTPGQRVTISC

SEQ ID NO: 547 - protein, 13 aa, Homo sapiens
SGSSSNIGSNTVN

SEQ ID NO: 548 - protein, 13 aa, Homo sapiens
SGSSSNIGSKTVN

SEQ ID NO: 549 - protein, 15 aa, Homo sapiens
WYQQLPGTAPKLLIY

SEQ ID NO: 550 - protein, 15 aa, Homo sapiens
WYQQFPGTAPKLLIY

SEQ ID NO: 551 - protein, 22 aa, Homo sapiens
SYVLTQPPSVSVAPGKTARITC

SEQ ID NO: 552 - protein, 22 aa, Homo sapiens
SYVLTQPPSVSVAPGQTARITC

SEQ ID NO: 553 - protein, 11 aa, Homo sapiens
GGNNIGSKSVH

SEQ ID NO: 554 - protein, 15 aa, Homo sapiens
WYQQKPGQAPVLVIY

SEQ ID NO: 555 - protein, 15 aa, Homo sapiens
WYQQKPGQAPVLVVY

SEQ ID NO: 556 - protein, 32 aa, Homo sapiens
GVPDRFSGSGSGTDFTLKISRVEAEDVGVYYC

SEQ ID NO: 557 - protein, 32 aa, Homo sapiens
GVPDRFSGSGSGTHLTLKISRVEAEDVGVYYC

SEQ ID NO: 558 - protein, 9 aa, Homo sapiens
MQALQTPLT

SEQ ID NO: 559 - protein, 10 aa, Homo sapiens
FGGGTKVEIK

SEQ ID NO: 560 - protein, 7 aa, Homo sapiens
WASTRES

SEQ ID NO: 561 - protein, 32 aa, Homo sapiens
GVPDRFSGSGSGTDFTLTISSLQAEDVAVYYC

SEQ ID NO: 562 - protein, 9 aa, Homo sapiens
QQYYSTPWT

SEQ ID NO: 563 - protein, 10 aa, Homo sapiens
FGQGTKVEIK

SEQ ID NO: 564 - protein, 7 aa, Homo sapiens
SNNQRPS

SEQ ID NO: 565 - protein, 7 aa, Homo sapiens
SNNRRPS

SEQ ID NO: 566 - protein, 32 aa, Homo sapiens
GVPDRFSGSKSGTSASLAISGLQSEDEADYYC

SEQ ID NO: 567 - protein, 10 aa, Homo sapiens
AAWDDSLNWV

SEQ ID NO: 568 - protein, 10 aa, Homo sapiens
ATWDDRLNWV

SEQ ID NO: 569 - protein, 10 aa, Homo sapiens
FGAGTKLTVL

SEQ ID NO: 570 - protein, 7 aa, Homo sapiens
YDSDRPS

SEQ ID NO: 571 - protein, 7 aa, Homo sapiens
DDSDRPS

SEQ ID NO: 572 - protein, 32 aa, Homo sapiens
GIPERFSGSNSGNTATLTISRVEAGDEADYYC

SEQ ID NO: 573 - protein, 32 aa, Homo sapiens
GIPERFSGSNSGNTATLTISRVEAGDEADYFC

SEQ ID NO: 574 - protein, 11 aa, Homo sapiens
QVWDSSSDPVV

SEQ ID NO: 575 - protein, 10 aa, Homo sapiens
FGGGTKLTVL

SEQ ID NO: 576 - protein, 127 aa, synthetic construct
  REGION 1..127: note = Synthetic
EMQLVESGGGLVQPGGSLRLSCAASGFTFSSHWMKWVRQAPGKGLEWVANINQDGSEKYYVDSVKGRFTISRDNAKNSLFLQMNSLRAEDTAVYYCARDIVLMVYDMDYYYYGMDVWGQGTTVTVSS

SEQ ID NO: 577 - protein, 112 aa, synthetic construct
  REGION 1..112: note = Synthetic
DIVMTQSPLSLPVTPGEPASISCRSSQSLLHSNGNNYLDWYLQKPGQSPQLLIYLGSNRASGVPDRFSGSGSGTDFTLKISRVEAEDVGVYYCMQTLQTPLTFGGGTKVEIK

SEQ ID NO: 578 - protein, 10 aa, Homo sapiens
GFTFSSHWMK

SEQ ID NO: 579 - protein, 17 aa, Homo sapiens
NINQDGSEKYYVDSVKG

SEQ ID NO: 580 - protein, 18 aa, Homo sapiens
DIVLMVYDMDYYYYGMDV

SEQ ID NO: 581 - protein, 16 aa, Homo sapiens
RSSQSLLHSNGNNYLD

SEQ ID NO: 582 - protein, 112 aa, synthetic construct
  REGION 1..112: note = Synthetic
  VARIANT 75: note = Xaa = H or D
  VARIANT 76: note = Xaa = F or L
  VARIANT 96: note = Xaa = T or A
DIVMTQSPLSLPVTPGEPASISCRSSQSLLHSNGNNYLDWYLQKPGQSPQLLIYLGSNRASGVPDRFSGSGSGTXXTLKISRVEAEDVGVYYCMQXLQTPLTFGGGTKVEIK

SEQ ID NO: 583 - protein, 127 aa, synthetic construct
  REGION 1..127: note = Synthetic
  VARIANT 31: note = Xaa = S or N
  VARIANT 35: note = Xaa = S or T
  VARIANT 58: note = Xaa = K or R
  VARIANT 69: note = Xaa = A or T
  VARIANT 74: note = Xaa = N or T
  VARIANT 76: note = Xaa = K or R
  VARIANT 80: note = Xaa = Y or F
  VARIANT 99: note = Xaa = D or P
  VARIANT 106: note = Xaa = D or A
  VARIANT 107: note = Xaa = I or L
  VARIANT 108: note = Xaa = D or H
  VARIANT 119: note = Xaa = Q or H
EVQLVESGGGLVQPGGSLRLSCAASGFTFSXYWMXWVRQAPGKGLEWVASIKQDGSEXYYVDSVKGRFXISRDXAXNSLXLQMNSLRAEDTAVYYCARXLVLMVYXXXYYYYGMDVWGXGTTVTVSS

SEQ ID NO: 584 - protein, 9 aa, synthetic construct
  REGION 1..9: note = Synthetic
  VARIANT 3: note = Xaa = T or A
MQXLQTPLT

SEQ ID NO: 585 - protein, 10 aa, synthetic construct
  REGION 1..10: note = Synthetic
  VARIANT 6: note = Xaa = S or N
  VARIANT 10: note = Xaa = S or T
GFTFSXYWMX

SEQ ID NO: 586 - protein, 17 aa, synthetic construct
  REGION 1..17: note = Synthetic
  VARIANT 9: note = Xaa = K or R
SIKQDGSEXYYVDSVKG

SEQ ID NO: 587 - protein, 18 aa, synthetic construct
  REGION 1..18: note = Synthetic
  VARIANT 1: note = Xaa = D or P
  VARIANT 8: note = Xaa = D or A
  VARIANT 9: note = Xaa = I or L
  VARIANT 10: note = Xaa = D or H
XLVLMVYXXXYYYYGMDV

SEQ ID NO: 588 - protein, 113 aa, synthetic construct [sequence omitted]

SEQ ID NO: 589 - protein, 118 aa, synthetic construct [sequence omitted]